European Patent Specification EP 3 279 323 B1, published March 8, 2023. Title: Amadoriase with improved specific activity. Applicant: Kikkoman Corporation. The sequence listing filed with the application follows.

SEQUENCE LISTING (248 sequences)

SEQ ID NO: 1 - protein, 437 aa, Coniochaeta sp. [sequence omitted]

SEQ ID NO: 2 - DNA, 1314 bp, Coniochaeta sp.
atgacgtcgaatcgtgcagatacaagggtgattgtcgtcggtggcggaggaacgattggttcctcgacagcgctgcatcttgtgaggagtggttatgctcccgcaaatatcacggtcttggacacatttgagattccatcggctcaatcagccggccatgatctcaacaagatcatgggaatacgactgcgcaacaaggtggacctgcaaatgagtctagaggctagacagatgtggaaggaggatgagttattccagcccttctttcacaataccggcagaatggactgcgaacacacgcctgagggtatcgaggacctgaaaaagcagtaccaggcactgcacgatgccggtgcgggtctggagaagactcatgcctggttggacaacgaggatgagatcttatccaagatgccgttgcttcaacgtgaccaaatacaaggatggaaagcaatatggagtcaagatggcggctggttagctgcggcaaaggccatcaatgcgatcggacagttcttgaaagaacgtggtgtaaagttcggattcggcggcgctggatccttcaagcaaccccttttcgacgatgaaggcacaacttgcattggcgttgagacggcagatggtaccaaatattacgctgacaaggtggtcttagcagctggcgcatggagcccaaccctggtggacctggaagatcaatgttgctcgaaggcttgggtgtatgctcatattcagttgacgcctgaagaggccgctgagtataagggtgtcccagttgtgtataatggcgaatttggcttcttctttgagcctgatgagtttggtgtaataaaggtgtgcgacgagttcccaggattctcgcgcttcaaggaacatcaaccctatggcgccccatctccgaaacggatatcagtaccacgatcgcacgccaagcatcccacagacacttatccagacgcatccgaagtcagcatcaaaaaagcaatcgcgacgtttctccctcgatttcaggacaaggagctcttcaatcgcgccttgtgctggtgtacagacactgcggacgctgctctcttgatgtgtgaacaccccaaatggaagaatttcattctagcgaccggcgacagcggacactcattcaaaatcttgcctaacgtcggaaaatacgtagtcgagttgatagagggccgcctgccggaggaaatggcttatcaatggaggtggcggccaggaggcgatgcactcaagtctagacgtgcggcaccgccaaaagatcttgcagacatgccaggatggaaacatgatccgaaattgtaa

SEQ ID NO: 3 - DNA, 30 bp, Artificial
  primer
tcatgggaatagcactgcgcaacaaggtgg

SEQ ID NO: 4 - DNA, 29 bp, Artificial
  primer
tattcccatgatcttgttgagatcatggc

SEQ ID NO: 5 - DNA, 29 bp, Artificial
  primer
acctgaaaaagctgtaccaggcactgcac

SEQ ID NO: 6 - DNA, 29 bp, Artificial
  primer
acctgaaaaagttctaccaggcactgcac

SEQ ID NO: 7 - DNA, 29 bp, Artificial
  primer
acctgaaaaagtattaccaggcactgcac

SEQ ID NO: 8 - DNA, 28 bp, Artificial
  primer
ctttttcaggtcctcgataccctcaggc

SEQ ID NO: 9 - DNA, 30 bp, Artificial
  primer
tcatgggaataaacctgcgcaacaaggtgg

SEQ ID NO: 10 - DNA, 30 bp, Artificial
  primer
tcatgggaatagatctgcgcaacaaggtgg

SEQ ID NO: 11 - DNA, 30 bp, Artificial
  primer
tcatgggaatacaactgcgcaacaaggtgg

SEQ ID NO: 12 - DNA, 30 bp, Artificial
  primer
tcatgggaatagaactgcgcaacaaggtgg

SEQ ID NO: 13 - DNA, 30 bp, Artificial
  primer
tgggaatagatctggccaacaaggtggacc

SEQ ID NO: 14 - DNA, 30 bp, Artificial
  primer
tgggaatagatctggaaaacaaggtggacc

SEQ ID NO: 15 - DNA, 30 bp, Artificial
  primer
tgggaatagatctgcacaacaaggtggacc

SEQ ID NO: 16 - DNA, 27 bp, Artificial
  primer
cagatctattcccatgatcttgttgag

SEQ ID NO: 17 - DNA, 28 bp, Artificial
  primer
tgagggtatcgaggccctgaaaaagctg

SEQ ID NO: 18 - DNA, 28 bp, Artificial
  primer
tgagggtatcgagaaactgaaaaagctg

SEQ ID NO: 19 - DNA, 28 bp, Artificial
  primer
tgagggtatcgagcgcctgaaaaagctg

SEQ ID NO: 20 - DNA, 28 bp, Artificial
  primer
ctcgataccctcaggcgtgtgttcgcag

SEQ ID NO: 21 - DNA, 30 bp, Artificial
  primer
aaaaagctgtaccagaaactgcacgatgcc

SEQ ID NO: 22 - DNA, 30 bp, Artificial
  primer
gcatcgtgcagtttctggtacagctttttc

SEQ ID NO: 23 - DNA, 30 bp, Artificial
  primer
aaaaagctgtaccagcgtctgcacgatgcc

SEQ ID NO: 24 - DNA, 30 bp, Artificial
  primer
gcatcgtgcagacgctggtacagctttttc

SEQ ID NO: 25 - DNA, 30 bp, Artificial
  primer
tcatgggaatagatgcgcgcaacaaggtgg

SEQ ID NO: 26 - DNA, 30 bp, Artificial
  primer
tcatgggaatagatgaccgcaacaaggtgg

SEQ ID NO: 27 - DNA, 30 bp, Artificial
  primer
tcatgggaatagatcatcgcaacaaggtgg

SEQ ID NO: 28 - DNA, 30 bp, Artificial
  primer
tcatgggaatagataagcgcaacaaggtgg

SEQ ID NO: 29 - DNA, 29 bp, Artificial
  primer
atctattcccatgatcttgttgagatcat

SEQ ID NO: 30 - DNA, 25 bp, Artificial
  primer
aggcgtgtgttcgcagtccattctg

SEQ ID NO: 31 - DNA, 30 bp, Artificial
  primer
gcgaacacacgcctaagggtatcgagaaac

SEQ ID NO: 32 - DNA, 29 bp, Artificial
  primer
acgtctagacttgagtgcatcgcctcctg

SEQ ID NO: 33 - DNA, 30 bp, Artificial
  primer
tcaagtctagacgtaaggcaccgccaaaag

SEQ ID NO: 34 - DNA, 30 bp, Artificial
  primer
acagacactgcggactctgctctcttgatg

SEQ ID NO: 35 - DNA, 28 bp, Artificial
  primer
gtccgcagtgtctgtacaccagcacaag

SEQ ID NO: 36 - protein, 436 aa, Aspergillus oryzae
MTVTKSSSILIIGAGTWGASTALHLGRRGYTNVTVLDPYTVPSAISAGNDVNKIISSGQYSNKKDEIEVNEILAEEAFKGWTTDPLFKPYYHDTGVVMSACSSAGLDRLGIRVRPEEEPDVSEVTKPEHFRQLAPAVLKGNFPGWRGYHIRSNAGWAHARNALVAAIREAEKLGVKFVTGTQGRVITLIFENNDVKGAVTADGKIWRAEQTVLCAGANAAQFLDFKDQLRPTAWTLAHIRLKPEERALYKNLPVIFNIEKGFFFEPDEERGEIKICDEHPGYTNMVKSADGHLTSLPFEKTQIPKESEARVRALLSETMPQLADRPFSFARVCWCADTANREFIIDRHPEHPSLVLGCGASGRGFKYLPSIGNLIVDAIEDKVPEKVHKLTRWSPDIAVDRKWRDTLGRFGGPNRVMDFHDVKEWTNVQNKDTAKL

SEQ ID NO: 37 - DNA, 1311 bp, Aspergillus oryzae
atgactgtcaccaaatcttcctcaatcctgatcatcggcgcaggcacttggggcgcttcaactgcccttcaccttggtcgcagaggatacaccaatgtcaccgtcctagacccttacacagtgccctcagcaatttcagctggaaatgacgtgaacaagatcatctcctcggggcaatacagcaacaaaaaggatgagattgaagttaacgaaattctcgccgaggaggcattcaaaggctggacaaccgaccctttgttcaagccatactaccacgacactggcgttgtaatgtctgcttgcagcagcgccggtctggatcgcctcggaatccgagtaaggccggaagaggaacctgatgtttccgaagtcacgaagccggagcacttccgccaactggcccccgctgtgctgaaaggaaacttcccggggtggagaggctaccacattcgttcgaacgctggctgggcgcacgcccgaaatgccctcgtggccgctatacgcgaagcagagaaacttggtgttaaattcgtaacaggcacccaaggaagagtcatcacccttatcttcgagaacaacgacgtcaagggcgcagtcaccgccgacggaaagatctggcgcgcggagcaaacagttctctgcgctggcgcaaatgctgcgcagttcttggattttaaggaccagctccgcccaacggcatggacactcgcccatatccggctcaaacctgaggaacgcgcgctctacaaaaacttgccggtgattttcaacattgagaaaggatttttcttcgagcctgatgaggagcgcggggagatcaagatctgcgacgaacatccgggatacactaacatggttaaatctgcggatggccacttgacgagtttgccctttgagaagacccagatccccaaggagtctgaagctagagtcagagctttactatcggagaccatgcctcaattagccgatcgcccatttagcttcgcccgcgtttgctggtgtgcggacaccgcaaaccgtgaattcatcattgaccgccaccctgaacacccgtctcttgttttgggatgcggtgcttccggaaggggtttcaaatatctcccctcaatcggcaacctcattgttgacgccattgaagacaaagtcccagagaaagttcacaagcttacgaggtggagtccagacattgctgttgacagaaagtggagggacactctggggcgctttggagggcctaaccgtgtcatggacttccatgatgtcaaggaatggactaacgtgcagaacaaggatactgcgaagctgtag

SEQ ID NO: 38 - protein, 437 aa, Phaeosphaeria nodorum
MAPSRANTSVIVVGGGGTIGSSTALHLVRSGYTPSNVTVLDAYPIPSSQSAGNDLNKIMGVSLRNPVDLQLALEARQMWNEDELFKKFFHNTGRLDCAHGEKDIADLKSGYQALVDAGLDATNEWLDSEDEILKRMPLLSRDQIKGWKAIFSKDGGWLAAAKAINAVGEYLRDQGVRFGFYGAGSFKAPLLAEGVCIGVETVDGTRYYADKVVLAAGAWSPTLVELHEQCVSKAWVYGHIQLTPEEAARYKNSPVVYNGDVGFFFEPNEHGVIKVCDEFPGFTRFKMHQPFGAKAPKRISVPRSHAKHPTDTIPDASDVSIRRAIATFMPQFKNKKMFNQAMCWCTDTADAALLICEHPEWKNFVLATGDSGHSFKLLPNIGKHVVELLEGTLADDLAHAWRWRPGSGDALKSRRSAPAKDLADMPGWNHDKPRANL

SEQ ID NO: 39 - DNA, 1314 bp, Phaeosphaeria nodorum
atggccccgtcgcgtgctaatacgtcggtcattgtggttggtggtggtggtacgattggctcatctacggctctgcatctggtccgctcaggctataccccgtcgaacgtgacggttctggatgcatacccgattccgagctctcagagcgctggcaacgacctgaataaaatcatgggtgtctctctgcgtaatccggtggatctgcagctggctctggaagcgcgccaaatgtggaacgaagacgaactgttcaagaagtttttccataacaccggccgtctggattgcgcgcacggtgaaaaagatattgccgacctgaagagcggctatcaggctctggtggatgcgggtctggacgccacgaacgaatggctggatagtgaagacgaaatcctgaaacgtatgccgctgctgtcccgcgatcaaattaaaggctggaaggcgatcttttcaaaagacggtggttggctggcagcagcaaaggcaattaatgcagttggtgaatatctgcgtgatcagggcgtccgcttcggtttttacggcgccggttctttcaaagcaccgctgctggctgaaggcgtctgcatcggtgtcgaaaccgtggatggcacgcgctattacgcagacaaagtggttctggctgcaggtgcatggtcgccgaccctggttgaactgcatgaacagtgtgtgagcaaagcgtgggtttacggccacattcaactgacgccggaagaagccgcacgttataagaacagcccggtcgtgtacaatggcgatgtgggctttttctttgaaccgaacgaacatggcgttatcaaagtctgcgatgaatttccgggttttacccgcttcaagatgcaccagccgtttggtgccaaagcaccgaagcgtattagtgtgccgcgctcccatgccaaacacccgaccgatacgatcccggatgcaagtgacgtttccattcgtcgcgctatcgcgacctttatgccgcagttcaagaacaaaaagatgttcaaccaagcgatgtgctggtgtaccgatacggccgacgctgcgctgctgatttgtgaacatccggaatggaaaaactttgttctggcgaccggcgattcaggtcattcgttcaaactgctgccgaatatcggcaagcacgttgtcgaactgctggagggtacgctggcagatgacctggcacacgcatggcgttggcgtccgggtagtggtgatgcactgaaaagccgtcgctctgctccggcgaaagacctggctgatatgccgggctggaaccatgacaaaccgcgtgctaatctgtaa

SEQ ID NO: 40 - protein, 437 aa, Eupenicillium terrenum
MAHSRASTKVVVVGGGGTIGSSTALHLIRSGYTPSNITVLDVYKTPSLQSAGHDLNKIMGIRLRNGPDLQLSLESLDMWQNDELFKPFFHQVGMIDCSSSKEGIENLRRKYQTLLDAGIGLEKTNVWLESEDEILAKAPNFTREQVKGWKGLFCTDGGWLAAAKAINAIGIFLQDKGVKFGFGDAGTFQQPLFAADGKTCIGLETTDGTKYFADKVVLAAGAWSPTLVDLEDQCVSKAWVFAHIQLTPKEADAYKNVPVVYDGEYGFFFEPDEYGVIKVCDEFPGFSRFKLHQPYGAASPKMISVPRSHAKHPTDTYPDASEVTIRKAIARFLPEFKDKELFNRTMCWCTDTADANLLICEHPKWKNFILATGDSGHSFKLLPNIGKYVVELLEGSLSQEMAGAWRWRPGGDALRSRRGAPAKDLAEMPGWKHDAHL

SEQ ID NO: 41 - DNA, 1314 bp, Eupenicillium terrenum
atggctcattcgcgtgcaagcaccaaagtcgtcgtggttgggggaggtggtacgatcgggtcttcgacggctctgcacttaatccgctctggatataccccctcaaatatcaccgtgcttgacgtatacaagaccccttcattgcaatctgcaggacatgatttgaacaagatcatgggcattcgattgcgcaacgggcctgacttgcagctttcgctggaatcactcgacatgtggcaaaacgatgagttgttcaagccattctttcaccaagtgggcatgattgattgttcgtcatccaaagagggtattgaaaatcttcgacgaaaataccagaccctcctcgatgcgggcattgggctggagaagacgaacgtttggctggaatctgaagatgagatcctcgccaaagcgccgaatttcacgcgtgaacaagtcaaggggtggaaaggcttattttgcactgatggaggctggcttgctgcagccaaggctatcaatgcgatcggaattttcctccaggacaaaggtgtcaagtttggctttggagatgctggtacctttcagcaacctctgttcgccgctgatggaaaaacttgcatcggacttgaaactacagacggaaccaagtactttgctgacaaggttgtcttggctgctggtgcgtggagtcccaccttggtggatctagaagatcagtgtgtttcaaaggcctgggttttcgctcatattcaactcacacccaaagaagcggacgcgtacaagaatgtgcctgtggtctatgatggtgaatatgggttctttttcgaacccgacgagtatggggtgatcaaagtctgtgacgagttccctggtttctctcgcttcaaactgcatcaaccgtacggggctgcatctcccaagatgatatccgtaccgcgatcacacgccaagcatcccacagatacctaccctgatgcctccgaagtcaccatacgcaaagcgatcgcaaggttcctgccagaatttaaagacaaggagctcttcaaccgtaccatgtgctggtgtacagatacggccgatgctaacttattgatttgcgaacacccgaagtggaagaatttcattctggccactggagatagcggacattccttcaagctgttgccaaacatcgggaaatacgtagttgagcttttagagggatctctatcgcaggaaatggctggtgcctggagatggagacccggaggtgatgctcttagatctagacgcggtgctccggcaaaggatcttgctgagatgccgggatggaagcatgatgcacatttgtga

SEQ ID NO: 42 - DNA, 30 bp, Artificial
  primer
aagatcatgggcattgatttgcgcaacggg

SEQ ID NO: 43 - DNA, 30 bp, Artificial
  primer
aatgcccatgatcttgttcaaatcatgtcc

SEQ ID NO: 44 - DNA, 30 bp, Artificial
  primer
gagggtattgaaaaacttcgacgaaaatac

SEQ ID NO: 45 - DNA, 26 bp, Artificial
  primer
ttcaataccctctttggatgacgaac

SEQ ID NO: 46 - DNA, 30 bp, Artificial
  primer
aaaaacttcgacgattataccagaccctcc

SEQ ID NO: 47 - DNA, 29 bp, Artificial
  primer
tcgtcgaagtttttcaataccctctttgg

SEQ ID NO: 48 - DNA, 30 bp, Artificial
  primer
cgacgattataccagaaactcctcgatgcg

SEQ ID NO: 49 - DNA, 30 bp, Artificial
  primer
ctggtataatcgtcgaagtttttcaatacc

SEQ ID NO: 50 - DNA, 30 bp, Artificial
  primer
agatacggccgattctaacttattgatttg

SEQ ID NO: 51 - DNA, 29 bp, Artificial
  primer
atcggccgtatctgtacaccagcacatgg

SEQ ID NO: 52 - DNA, 30 bp, Artificial
  primer
tcatgggcattgatcatcgcaacgggcctg

SEQ ID NO: 53 - DNA, 29 bp, Artificial
  primer
atcaatgcccatgatcttgttcaaatcat

SEQ ID NO: 54 - protein, 441 aa, Neocosmospora vasinfecta
MTTPRKETTVLIIGGGGTIGSSTALHLLRAGYTPSNITVLDTYPIPSAQSAGNDLNKIMGIRLRNKVDLQLSLEARDMWRNDALFRPFFHNTGRLDCESSAEGVEGLRREYQKLVEAGVGLEETHEWLDSEEAILEKAPLLQREEIEGWKAIWSEEGGWLAAAKAINAIGEELQRQGVRFGFGGAGSFKRPLFADDGTTCIGVETVDGTQYHADKVVLAAGAWSPALVDLEEQCCSKAWVYAHMQLTPEEAAVYKGCPVVYHGDVGFFFEPNENGVIKVCDEFPGFTRFKQHQPYGAPAPKPVSVPRSHAKHPTDTYPDASEESIKRAVSTFLPRFKDKPLFNRALCWCTDTADSALLICEHPRWKNFILATGDSGHSFKLLPIIGKHVVELVEGRLADDLAEAWRWRPGQGDARKSIRAAPAKDLADMPGWKHDQDSESR

SEQ ID NO: 55 - DNA, 1326 bp, Neocosmospora vasinfecta
atgacgaccccgcgtaaagaaacgacggtcctgattattggtggtggtggcacgattggtagctcgacggctctgcatctgctgcgtgccggctataccccgtctaacattaccgtgctggatacgtacccgatcccgagtgcccagtccgcaggcaacgacctgaataaaattatgggtatccgtctgcgcaataaagttgatctgcaactgagcctggaagcccgtgatatgtggcgcaacgacgcactgtttcgtccgtttttccataataccggccgcctggactgcgaaagctctgctgaaggcgtggaaggtctgcgtcgcgaatatcagaaactggtggaagcaggcgttggtctggaagaaacgcacgaatggctggatagcgaagaagctattctggaaaaagcgccgctgctgcaacgtgaagaaattgaaggttggaaagccatctggtctgaagaaggcggttggctggcggccgcaaaagctattaacgcgatcggcgaagaactgcagcgtcaaggcgttcgcttcggttttggcggtgccggtagttttaaacgcccgctgttcgcagatgacggcaccacgtgtatcggtgtcgaaaccgtggatggcacgcagtatcatgcggacaaagtggttctggctgcaggtgcttggtcaccggcgctggtcgatctggaagaacagtgctgttcgaaagcctgggtgtacgcacacatgcaactgaccccggaagaagccgcagtttataaaggctgcccggtcgtgtaccacggcgatgtcggctttttctttgaaccgaacgaaaatggcgttattaaagtctgtgacgaattcccgggttttacgcgtttcaaacagcatcaaccgtatggtgccccggcaccgaaacctgtgagtgttccgcgctcccatgcgaaacacccgaccgatacgtacccggacgcttcagaagaatcgatcaaacgtgccgtgagtacctttctgccgcgcttcaaagataaaccgctgtttaaccgtgcactgtgctggtgtaccgatacggccgactccgcactgctgatttgcgaacacccgcgctggaaaaattttatcctggcgaccggcgatagcggtcattctttcaaactgctgccgattatcggcaaacacgttgtcgaactggttgaaggtcgtctggcggatgacctggctgaagcgtggcgttggcgtccgggtcagggtgatgcacgtaaaagcattcgcgctgcgccggcgaaagacctggcggatatgccgggctggaaacacgaccaagactcggaatcacgctga

SEQ ID NO: 56 - DNA, 29 bp, Artificial
  primer
ttatgggtatcgatctgcgcaataaagtt

SEQ ID NO: 57 - DNA, 30 bp, Artificial
  primer
gctcagttgcagatcaactttattgcgcag

SEQ ID NO: 58 - DNA, 30 bp, Artificial
  primer
gaaggcgtggaaaaactgcgtcgcgaatat

SEQ ID NO: 59 - DNA, 30 bp, Artificial
  primer
ttccaccagtttctgatattcgcgacgcag

SEQ ID NO: 60 - DNA, 27 bp, Artificial
  primer
ctgcgtcgcctgtatcagaaactggtg

SEQ ID NO: 61 - DNA, 30 bp, Artificial
  primer
accaacgcctgcttccaccagtttctgata

SEQ ID NO: 62 - protein, 438 aa, Aspergillus nidulans
MTPRANTKIIVVGGGGTMGSSTALHLLRAGYTPSNITVLDTCPIPSAQSAGYDLNKIMGIRLRNKPDLQLSLEALDMWKNDPLFKPFFHNVGMIDVSSTEEGIEGLRKKYQSLLDAGIGLEKTNFMLESEDEILAKAPHFTQEQIKGWKGLFCGDGGWLAAAKAINAIGQFLKEQGVKFGFGGAGTFKKPLFADAHEKTCIGVETVDGTKYYADKVVLAAGAWSSTLVDLEEQCVSKAWVFAHIQLTPAEAAAYKNTPVIYDGDYGFFFEPNENGIIKVCDEFPGFTHFKMHQPYGSPAPKPISVPRSHAKHPTDTYPHASEVTIKKAINRFLPRFNDKELFNRAMCWCTDTADANLLVCEHPRWKGFYLATGDSGHSFKLLPNIGKHVVELLEERLESVFKDAWRWRPGSGDALKSRRAAPAKDLADMPGWRNEAKM

SEQ ID NO: 63 - DNA, 1317 bp, Aspergillus nidulans
atgacgccccgagccaacaccaaaatcattgtcgtcggcggcggcggcacaatgggctcgtcgacagccctacacctcctgcgcgccggctacacgccgtccaacattacagtgctcgacacgtgccctatcccctccgcacagtctgcaggctacgacctgaacaaaatcatggggatccgtctgcgcaacaagcctgatttacagctctctcttgaggcgctggacatgtggaaaaatgatcctctcttcaagccgtttttccacaatgttggaatgatcgacgtctcttcaacagaggaaggcatcgagggtcttcggaagaaataccagtctcttctcgacgcaggcattgggctcgagaagacgaatttcatgctggaaagtgaagacgagatcctggctaaagcgccgcatttcacgcaggagcagattaaaggctggaaaggcctgttctgtggcgacggcggctggctcgctgcagccaaagccatcaatgccattgggcagttcctcaaggaacagggcgtcaagtttggattcggcggcgccggcacgttcaaaaagccactcttcgccgatgcccacgagaagacgtgcatcggcgtcgagactgtagacggcacaaagtactacgccgacaaggtcgttctagcagctggtgcctggagttcgacgttggtcgatctggaggagcagtgcgtttcaaaggcctgggtctttgcccacatccaactgacgcccgctgaagcagccgcgtataagaacactcctgttatatacgacggtgactatgggtttttctttgagccgaatgaaaacggcatcataaaagtctgtgacgaattccctggcttcacgcatttcaaaatgcaccagccgtacggctcgccggcgcccaaacccatctctgtgcctcgttcccatgcgaagcaccccacagatacatacccgcacgcgtcggaggtcacgatcaaaaaggctatcaaccggttcctgccgaggttcaatgacaaggaactgtttaacagggccatgtgctggtgcaccgataccgcggatgcaaatctgcttgtttgtgagcatccacgctggaaggggttttatcttgcaacaggggacagtgggcattcgttcaagttgctgccgaatattggaaagcatgttgtcgagttattggaggagaggctggaaagtgtgtttaaggatgcttggaggtggaggcctggcagtggggatgcattaaaaagtagacgggctgcgcctgcgaaggacctggcggatatgccggggtggaggaatgaggcaaagatgtag

SEQ ID NO: 64 - DNA, 30 bp, Artificial
  primer
atcatgggcatcgatctgcgcaacaagcct

SEQ ID NO: 65 - DNA, 30 bp, Artificial
  primer
agagagctgtaaatcaggcttgttgcgcag

SEQ ID NO: 66 - DNA, 30 bp, Artificial
  primer
gaaggcatcgagaaacttcggaagaaatac

SEQ ID NO: 67 - DNA, 30 bp, Artificial
  primer
gtcgagaagagactggtatttcttccgaag

SEQ ID NO: 68 - DNA, 27 bp, Artificial
  primer
cttcggaagctgtaccagtctcttctc

SEQ ID NO: 69 - DNA, 30 bp, Artificial
  primer
cccaatgcctgcgtcgagaagagactggta

SEQ ID NO: 70 - DNA, 30 bp, Artificial
  primer
cttctcgagcccaatgcctgcgtcgagaag

SEQ ID NO: 71 - DNA, 30 bp, Artificial
  primer
gataccgcggatagcaatctgcttgtttgt

SEQ ID NO: 72 - DNA, 30 bp, Artificial
  primer
ccagcgtggatgctcacaaacaagcagatt

SEQ ID NO: 73 - DNA, 30 bp, Artificial
  primer
atcatgggcatcgatcatcgcaacaagcct

SEQ ID NO: 74 - DNA, 27 bp, Artificial
  primer
agagagctgtaaatcaggcttgttgcg

SEQ ID NO: 75 - DNA, 30 bp, Artificial
  primer
tcttcaacagagaaaggcatcgagaaactt

SEQ ID NO: 76 - DNA, 27 bp, Artificial
  primer
gtacagcttccgaagtttctcgatgcc

SEQ ID NO: 77 - DNA, 29 bp, Artificial
  primer
atcatgggtgtcgatctgcgtaatccggt

SEQ ID NO: 78 - DNA, 30 bp, Artificial
  primer
agccagctgcagatccaccggattacgcag

SEQ ID NO: 79 - DNA, 30 bp, Artificial
  primer
aaagatattgccaaactgaagagcggctat

SEQ ID NO: 80 - DNA, 30 bp, Artificial
  primer
atccaccagagcctgatagccgctcttcag

SEQ ID NO: 81 - DNA, 27 bp, Artificial
  primer
ctgaagagcctgtatcaggctctggtg

SEQ ID NO: 82 - DNA, 30 bp, Artificial
  primer
gtccagacccgcatccaccagagcctgata

SEQ ID NO: 83 - DNA, 30 bp, Artificial
  primer
agcctgtatcagaaactggtggatgcgggt

SEQ ID NO: 84 - DNA, 30 bp, Artificial
  primer
gttcgtggcgtccagacccgcatccaccag

SEQ ID NO: 85 - DNA, 30 bp, Artificial
  primer
gatacggccgacagcgcgctgctgatttgt

SEQ ID NO: 86 - DNA, 30 bp, Artificial
  primer
ccattccggatgttcacaaatcagcagcgc

SEQ ID NO: 87 - DNA, 29 bp, Artificial
  primer
atgggtgtcgatcatcgtaatccggtgga

SEQ ID NO: 88 - DNA, 30 bp, Artificial
  primer
cagagccagctgcagatccaccggattacg

SEQ ID NO: 89 - protein, 443 aa, Cryptococcus neoformans
MPPSRASTKVIVIGGGGTLGSSTALHLLRAGYTPSNITVLDTYLIPSAQSAGNDLNKIMGIRIRNPVDKQLSLEARDMWRNDEVFKPYFHNTGRLDCAHTPESIASLRKSYEAILKAGSGLEKTHHWLSTEDEILARAPLLDRKQIKGWKAIYSEDGGWLAAAKAINSIGQVLKEKGVTFGFGSAGSFKKPLFDEDGTKAIGIETVDGTQYFADKVVLAAGAWSPTLVDLEGQCCSKAWVYAHMQLTPEEAAEYKECPVVYNSELGFFFEPNEKGVIKVCDEFPGFTRFKQHQPYGASSTKHISFPRSHAKHPTDTIPDESDASIRRAISAFLPRFKEKELFNRALCWCTDTADANLLICEHPKWKNFILATGDSGHSFKILPNIGKHVVELIEGTLAEDLAESWRWRPGSGDPLISRRAAPARDLADLPGWNHDEPSDDDMD

SEQ ID NO: 90 - DNA, 1332 bp, Cryptococcus neoformans
atgccgccgtcccgtgcttcaacgaaagtgattgtcattggtggtggtggtacgctgggctcctcaaccgccctgcatctgctgcgcgcgggctataccccgagtaacattaccgtgctggatacgtacctgatcccgagtgcccagtccgcaggcaacgacctgaataaaattatgggtattcgtatccgcaatccggtggataaacaactgagcctggaagcccgtgatatgtggcgcaacgacgaagttttcaaaccgtacttccataacaccggtcgtctggactgcgctcacacgccggaatcaattgcgtcgctgcgtaaaagctacgaagccatcctgaaagcaggctcaggtctggaaaaaacccatcactggctgtcgacggaagatgaaatcctggcacgtgcaccgctgctggaccgtaaacagattaaaggttggaaagcaatctatagtgaagatggcggttggctggcggccgcaaaagctattaactccatcggccaagtcctgaaagaaaaaggtgtgaccttcggctttggtagcgcaggctcttttaaaaaaccgctgttcgatgaagacggcacgaaagccattggtatcgaaaccgttgatggtacgcagtattttgccgacaaagtggttctggctgcaggtgcatggagcccgaccctggttgatctggaaggccagtgctgttctaaagcttgggtctacgcgcacatgcaactgacgccggaagaagccgcagaatataaagaatgcccggtcgtgtacaacagcgaactgggctttttctttgaaccgaacgaaaaaggtgtgatcaaagtttgtgatgaattcccgggctttacccgtttcaaacagcatcaaccgtacggtgctagctctacgaaacacattagctttccgcgctctcatgcgaaacacccgaccgatacgatcccggatgaaagtgacgcctccattcgtcgcgctatctctgcgtttctgccgcgtttcaaagaaaaagaactgtttaaccgcgcgctgtgctggtgtaccgatacggctgacgcgaacctgctgatttgtgaacacccgaaatggaaaaattttatcctggccaccggcgattcaggtcattcgttcaaaattctgccgaatatcggcaaacacgttgtcgaactgattgaaggtaccctggccgaagatctggcagaaagctggcgttggcgtccgggcagtggtgacccgctgatctcccgtcgcgctgcgccggcgcgcgacctggcggacctgccgggctggaaccacgacgaaccgagcgacgatgacatggactga

SEQ ID NO: 91 - DNA, 30 bp, Artificial
  primer
attatgggtattgatatccgcaatccggtg

SEQ ID NO: 92 - DNA, 30 bp, Artificial
  primer
gctcagttgtttatccaccggattgcggat

SEQ ID NO: 93 - DNA, 30 bp, Artificial
  primer
gaatcaattgcgaaactgcgtaaaagctac

SEQ ID NO: 94 - DNA, 30 bp, Artificial
  primer
tttcaggatggcttcgtagcttttacgcag

SEQ ID NO: 95 - DNA, 30 bp, Artificial
  primer
ctgcgtaaactgtacgaagccatcctgaaa

SEQ ID NO: 96 - DNA, 30 bp, Artificial
  primer
acctgagcctgctttcaggatggcttcgta

SEQ ID NO: 97 - DNA, 30 bp, Artificial
  primer
aaactgtacgaaaaaatcctgaaagcaggc

SEQ ID NO: 98 - DNA, 30 bp, Artificial
  primer
tttttccagacctgagcctgctttcaggat

SEQ ID NO: 99 - protein, 440 aa, Curvularia clavata
MAPSRANTSVIVVGGGGTIGSSTALHLVRSGYTPSNITVLDAYPIPSSQSAGNDLNKIMGIRLRNKVDLQLSLEARQMWREDDLFKEYFHNTGRLDCAHGEEGLADLRQAYQALLDANAGLEETTEWLDSEDEILKKMPLLSRDQIKGWKAVYSQDGGWLAAAKAINAIGEYLRAQGVKFGFGGAGSFKQPLLAEGVCIGVETVDGTRYYADKVVLAAGAWSPTLVELHEQCVSKAWVYGHIQLTPEEAAEYKNSPVVYNGDVGFFFEPNEHGVIKVCDEFPGFTRFKMHQPFGAKAPKRISVPRSHAKHPTDTIPDASEKSIRKAIATFLPKFTEKELFNRHLCWCTDTADAALLICEHPEWKNFVLATGDSGHSFKLLPNIGKHVVELLEGTLADDLAHAWRWRPGSGDALKSRRSAPAKDLADMPGWKHDDVVKSKL

SEQ ID NO: 100 - DNA, 1323 bp, Curvularia clavata
atggccccgtcgcgtgctaatacgtcggtcattgtggttggtggtggtggtacgattggctcatctacggctctgcatctggtccgctcaggctataccccgtcgaacattacggttctggatgcatacccgattccgagctctcagagcgctggcaacgacctgaataaaatcatgggtatccgtctgcgtaataaggtggatctgcagctgtctctggaagcgcgccaaatgtggcgcgaagacgatctgttcaaggagtatttccataacaccggccgtctggattgcgcgcacggtgaagaaggtcttgccgacctgcgtcaagcctatcaggctctgctggatgcgaatgcgggtctggaagagacgaccgaatggctggatagtgaagacgaaatcctgaaaaaaatgccgctgctgtcccgcgatcaaattaaaggctggaaggcggtgtattcacaggacggtggttggctggcagcagcaaaggcaattaatgcaattggtgaatatctgcgtgctcagggcgtcaaattcggttttggcggcgccggttctttcaaacaaccgctgctggctgaaggcgtctgcatcggtgtcgaaaccgtggatggcacgcgctattacgcagacaaagtggttctggctgcaggtgcatggtcgccgaccctggttgaactgcatgaacagtgtgtgagcaaagcgtgggtttacggccacattcaactgacgccggaagaagccgcagaatataagaacagcccggtcgtgtacaatggcgatgtgggctttttctttgaaccgaacgaacatggcgttatcaaagtctgcgatgaatttccgggttttacccgcttcaagatgcaccagccgtttggtgccaaagcaccgaagcgtattagtgtgccgcgctcccatgccaaacacccgaccgatacgatcccggatgcaagtgaaaaatccattcgtaaagctatcgcgacctttctgccgaagttcacggagaaagagctgttcaaccgtcatctgtgctggtgtaccgatacggccgacgctgcgctgctgatttgtgaacatccggaatggaaaaactttgttctggcgaccggcgattcaggtcattcgttcaaactgctgccgaatatcggcaagcacgttgtcgaactgctggagggtacgctggcagatgacctggcacacgcatggcgttggcgtccgggtagtggtgatgcactgaaaagccgtcgctctgctccggcgaaagacctggctgatatgccgggctggaaacatgacgatgtggtgaaaagcaaactgtaa

SEQ ID NO: 101 - DNA, 30 bp, Artificial
  primer
atcatgggtatcgatctgcgtaataaggtg

SEQ ID NO: 102 - DNA, 30 bp, Artificial
  primer
cagagacagctgcagatccaccttattacg

SEQ ID NO: 103 - DNA, 30 bp, Artificial
  primer
gaaggtcttgccaaactgcgtcaagcctat

SEQ ID NO: 104 - DNA, 30 bp, Artificial
  primer
atccagcagagcctgataggcttgacgcag

SEQ ID NO: 105 - DNA, 30 bp, Artificial
  primer
cttgccaaactgcgtcaactgtatcaggct

SEQ ID NO: 106 - DNA, 30 bp, Artificial
  primer
acccgcattcgcatccagcagagcctgata

SEQ ID NO: 107 - DNA, 30 bp, Artificial
  primer
cgtcaactgtatcagaaactgctggatgcg

SEQ ID NO: 108 - DNA, 30 bp, Artificial
  primer
ctcttccagacccgcattcgcatccagcag

SEQ ID NO: 109 - DNA, 30 bp, Artificial; identical to SEQ ID NO: 85
  primer

SEQ ID NO: 110 - DNA, 30 bp, Artificial; identical to SEQ ID NO: 86
  primer

SEQ ID NO: 111 - DNA, 30 bp, Artificial
  primer
atcatgggtatcgatcatcgtaataaggtg

SEQ ID NO: 112 - DNA, 30 bp, Artificial
  primer
aagctgtaccagaaacttctcgacgcaggc

SEQ ID NO: 113 - protein, 440 aa, Pyrenochaeta sp.
MAASRAKTTVIVVGGGGTIGSSTALHLLRSGYTPSNITVLDTYPIPSLQSAGNDLNKIMGIRLRNKVDLQLSLEAREMWREDELFRDFFHNTGRLDCAHGEKGINDLRQAYQTLLDANAGLEETNEWLDSEDEILARMPLLSREQIKGWKAVFSRDGGWLAAGKAINAIGEYLRKEGVKFGFGGAGSFQQPLLAEGICIGVETTDGTRYYADKVVLAAGAWSPALVDLEDQCVSKAWVYAHMQLTPKEAAAYKDTPVVYNGDLGFFFEPNEHGVIKVCDEFPGFTRFKKHQPFGARAPKRISVPRSHAKHPTDTYPHASEASIKKAIAAFLPQFKDKELFNRAMCWCTDTADAALLICEHPQWKNFMLATGDSGHSFKLLPNIGKHVVELIEGTLAADLAHAWRWRPGIGDALQSRRAAPAKDLADMPGWNHDESPRAKL

SEQ ID NO: 114 - DNA, 1323 bp, Pyrenochaeta sp.
atggccgcttcacgagcaaagacgacagtgatcgtcgtgggtggcggcggtaccattgggtcatcaacagcgctccaccttctacgttcaggttatactccatcgaatatcacagttttggacacatatccaattccttcattacagtccgcgggcaatgatttaaacaagattatgggcattcgcttgcgaaacaaagtcgacctccaattgagtttagaggctagggagatgtggagagaagatgaactttttagagatttttttcacaatactgggcgactggattgtgcccatggcgaaaaaggaatcaatgatcttaggcaggcatatcaaacactactcgacgccaatgccggtttggaagagacgaacgagtggctggactctgaggacgaaattctggcaagaatgccgctcttgagtcgagagcagatcaagggctggaaagcggtcttcagccgagacggcggttggctcgccgcaggtaaggccatcaatgcaattggcgagtatctgcgcaaggaaggagtcaagtttggctttggcggcgcgggatcgttccagcagccgcttcttgcagagggtatttgcattggcgtggaaacaacggatggaactagatactacgccgacaaagttgtcctggcagctggtgcatggagtcctgcattggtggacttggaagaccagtgtgtttcaaaagcatgggtctatgctcacatgcagctcaccccgaaggaggctgcggcatacaaagacacaccagtagtctacaatggcgatctgggatttttctttgaaccaaacgagcatggcgtgatcaaagtctgcgacgagttcccaggcttcacacgttttaagaagcatcaaccatttggtgcaagggcaccaaaacggatatcggttcccagatctcatgccaaacaccctactgatacttatcctcacgcatccgaagccagtatcaagaaagctattgcggcattcttaccacagttcaaggacaaggagctgttcaaccgcgcaatgtgctggtgcacagatacagctgatgcagccttgttgatctgcgaacacccgcaatggaagaatttcatgcttgctactggagacagcgggcactcatttaagctcttaccaaatatcggcaagcatgtagttgaactgattgaaggcactctggcggcagatcttgcccatgcttggaggtggcgacctgggattggtgacgctttgcagtcaaggcgagcggcacctgcgaaggatctggcggacatgccaggatggaatcatgatgaatctcctagggcgaaattgtaa

SEQ ID NO: 115 - protein, 452 aa, Arthrinium sp.
MAASRKTTKVIVVGGGGTIGSSTALHLLRSGYTATNITVLDTYPIPSAQSAGNDLNKIMGIRLRNPVDKQLSLEAQDMWCHDELFKPYFHNTGRMDCEGTEKGIAALKQQYQTLLDADVGLEKTTEWLDSEDAILAKMPLLERDQIKGWKAIFSQDGGWLAAAKAINAIGEELKRQGVNFGFGGAGAFKKPLFAPDGSTCIGVETVDGTKYYGDKVVLAAGAWSPALVDLEEQCCSKAWVYAHMQLTPHEAAEYQGCPVVYHGDLGFFFEPNEHGVIKVCDEFPGFTRFLEQHQSYGAPAPTRVSVPRSHAKHPTDTYPDASEQSIRRAVAAFLPRFQSKELFNRAMCWCTDTADAALLICEHPRWRNFILATGDSGHSFKLLPNIGKHVVELLEGRLADDLAQAWRWRPGQGDALKSRRAAPAKDLADMPGWNHDGDSGNATSGTSSEHKL

SEQ ID NO: 116 - DNA, 1359 bp, Arthrinium sp.
atggcggcgtcacgaaagaccaccaaagtgattgtcgtgggcggcggaggcaccatcggctcatccacggctctacatcttctccggtcggggtatacggccaccaacattaccgtcctggacacctaccccatcccctcggcgcagtcggccggcaacgacctgaacaagattatggggatccgcctgcggaacccggtcgacaagcagctcagccttgaagcccaggacatgtggtgccatgacgagctcttcaagccctacttccacaacaccggcaggatggactgcgagggcaccgagaagggcatcgcggcgctcaagcagcagtaccagaccttgcttgacgccgacgtgggcctcgagaagacgacggagtggctcgacagtgaggatgccatcctggcaaagatgccactcctggagcgcgaccaaatcaaaggatggaaagcgatatttagccaggacggcggttggctggccgcagctaaagccatcaacgcgataggcgaggaactgaagaggcagggcgtcaacttcgggttcggcggggcgggcgccttcaagaagccccttttcgccccggacggatccacctgcatcggcgtcgagacggtggatggaaccaagtactacggcgacaaggtcgtcctggccgcgggcgcgtggagccctgcgctggtcgacctggaagagcagtgctgctccaaggcctgggtgtacgcccacatgcagctgacgccgcacgaggcagccgagtaccagggctgtccggtcgtgtaccacggcgacctcggcttcttcttcgagcccaacgagcacggcgtcatcaaggtgtgcgacgagttccccggcttcacgcggttcctcgagcagcaccagtcgtacggcgcgccggcgccgacgcgcgtctcggtgccccggtcgcacgcgaagcaccccaccgacacatacccggacgcgtcggagcagtcgatccggcgggccgtggccgcgttcctgccgcgattccaaagcaaagagcttttcaaccgcgccatgtgctggtgcaccgacacggccgacgccgcgctgctgatctgcgagcacccccgctggcgcaattttattctggctacgggcgacagcggacactcgttcaagctcctgcccaacatcggcaagcacgtggtcgagctgctggaaggccggctagcggatgacctggcgcaggcgtggaggtggcgccccggtcagggggatgcgttgaagtctagacgggcggctccggctaaggatctggcggatatgccagggtggaatcatgacggggattcagggaatgctacgtctggaacaagctcggagcacaaattgtag

SEQ ID NO: 117 - protein, 440 aa, Curvularia clavata
MAPSRANTSVIVVGGGGTIGSSTALHLVRSGYTPSNITVLDTYPIPSAQSAGNDLNKIMGIRLRNKVDLQLSLEARQMWREDDLFKEYFHNTGRLDCAHGEEGLADLRQAYQALLDANAGLEETTEWLDSEDEILKKMPLLDREQIKGWKAVYSQDGGWLAAAKAINAIGEYLRAQGVKFGFGGAGSFKQPLLAEGVCIGVETVDGTRYYADKVVLAAGAWSPVLVDLEDQCVSKAWVYAHIQLTPEEAAEYKNVPVVYNGDVGFFFEPDEHGVIKVCDEFPGFTRFKQHQPYGAKAPKRISVPRSAAKHPTDTYPDASEKSIRKAIATFLPKFTEKELFNRHLCWCTDTADAALLMCEHPEWKNFVLATGDSGHTFKLLPNIGKHVVELLEGTLAEDLAHAWRWRPGTGDALKSRRAAPAKDLADMPGWKHDDVVKSKL

SEQ ID NO: 118 - DNA, 1323 bp, Curvularia clavata
atggcgccctcaagagcaaacacttctgttatcgttgtcggtggcggtggcactattggctcttcaaccgctcttcatctagtccgctcgggctacacaccatctaacatcaccgttcttgacacataccctatcccatcagcgcagtcagctggaaatgacctgaataagatcatgggtatccgcttgcggaacaaggtcgatctccaattgagtctagaagccaggcagatgtggagagaggatgacctattcaaagagtatttccacaacactggaagactcgactgtgcacatggggaagagggacttgcagatttgagacaggcataccaggctctgctcgacgctaacgcgggtctcgaagaaacaacagaatggcttgactccgaagacgaaattctaaagaaaatgccgcttctggaccgcgagcaaatcaagggctggaaagcggtttacagccaagacggcggctggctggctgcagcaaaagccatcaatgctataggcgagtacttgcgagcccaaggagttaagtttggttttggtggtgctggatcgttcaagcagcctcttttggccgagggagtgtgcattggcgtagagacagtcgacgggacgaggtactacgccgataaagttgtgcttgcagctggtgcttggagtccggtattggtcgacctggaagatcaatgcgtttcaaaagcttgggtatatgctcacatacagcttacgcctgaggaagcagcagagtacaaaaacgtgcctgtggtatacaacggcgacgtcggcttcttcttcgagcctgacgagcacggcgttatcaaggtttgtgacgaatttccaggttttacacgcttcaagcaacatcagccatatggcgccaaagcaccgaaacgtatctccgtgcccagatcggcagcgaagcacccgacggatacttaccccgatgcgtcggagaagagcatccgcaaggccattgcaactttcctgcccaagttcacagagaaggagctattcaaccggcatctatgttggtgtacggatacggctgacgctgcgctattgatgtgtgagcatcccgagtggaagaactttgtgctggcgacaggggacagcgggcacacattcaaacttttgccaaatatcggcaagcatgtggttgagcttctcgagggtacactcgcggaggatctggcacatgcatggagatggcggcctggtactggcgatgcgctgaaatcaagaagagcggcaccggcgaaggatttagcagatatgcctggctggaagcatgacgatgttgtcaagtccaagttatag

SEQ ID NO: 119 - protein, 438 aa, Emericella nidulans
MAPRANTKIIVVGGGGTMGSSTALHLLRAGYTPSNITVLDTYPIPSAQSAGYDLNKIFGIRLRNKPDLQLYLEALDMWKNDPLFKPFFHNVGQMDVSSTEEGIKKLRMRYQSLLDAGIGLEKTNFLLESEDEILAKAPHFTREQIKGWKGLFCGDGGWLAAAKAINAIGQFLKEQGVKFGFGEAGTFKKPLFADADEKTCIGVETVDGTKYYADKVVLAAGAWSSTLVDLEEQCVSKAWVFAHIQLTPAEAAAYKNTPVIYDGDYGFFIEPDENGIIKVCDEFPGFTHFKMHQPYGSPVPKLISVPRSHAKHPTDTYPHASEVTIKKAINRFLPRFNDKELFNRAMCWCTDTADANLLVCEHPRWKGFYLATGDSGHSFKLLPNIGKHVVELLEGRLESVFKDAWRWRPGSGDALKSRRAAPAKDLADMPGWRNEAKM

SEQ ID NO: 120 - DNA, 1317 bp, Emericella nidulans
atggcgccccgagccaacaccaaaatcatcgtcgtcggcggcggcggcacaatgggctcgtcgacagccctacacctcctgcgcgccggctacacgccgtccaacatcacagtgctcgacacgtaccctatcccttccgcacagtctgcaggctacgacctgaacaaaatcttcggcatcaggctgcgcaacaagcctgacttacaactctatcttgaggcgctggacatgtggaaaaatgatcctctattcaagccgtttttccacaatgttggacagatggacgtctcttcaacagaagaaggcatcaaaaagcttcgcatgagataccagtctcttctcgacgcaggcattgggctcgagaagacgaatttcctgctggaaagtgaagacgagatcctggctaaagcgccgcatttcacgcgggagcagattaaaggctggaaagggctgttctgtggcgacggcggttggctcgctgcagccaaagccatcaatgccatcgggcagttcctcaaggaacagggcgtcaagtttggatttggcgaggccggcacgttcaaaaagccactcttcgccgatgccgacgagaagacgtgcatcggcgtcgaaactgtagacggcacaaaatactacgccgacaaggtcgttctagcagctggtgcctggagttcgacgttggtcgatctggaggagcagtgcgtttcaaaggcctgggtctttgcccacatccaactgacgcccgctgaagcagccgcgtacaagaacactcctgttatatacgacggtgactatgggtttttcattgagccggacgagaacggcatcataaaagtctgcgacgaattccctggcttcacgcacttcaagatgcaccagccgtacggctcaccggtgcccaaattgatctctgtgcctcgctcccatgcgaagcaccccacagatacatacccgcacgcgtcggaggtcaccatcaaaaaggctatcaaccggttcctgccgaggttcaatgacaaggaactgtttaacagggccatgtgctggtgcaccgataccgcggatgcaaatctgcttgtttgtgagcatccacgctggaaggggttttatcttgcaacaggggacagcgggcattcgttcaagttgctgccgaatattggaaagcacgttgtcgagttattggaggggaggctggaaagtgtgtttaaggatgcttggaggtggaggcctggcagtggggatgcattaaagagtagacgggctgcgcctgcgaaggacctggcggatatgccggggtggaggaatgaggcaaagatgtag

SEQ ID NO: 121 - protein, 441 aa, Ulocladium sp.
MAPNRANISVIVVGGGGTIGSSTALHLVRSGYTPSNITVLDTYPIPSAQSAGNDLNKIMGIRLRNKVDLQLSLEARQMWTEDDLFKEYFHKTGRLDCAHGEKGLADLKQAYQALLDANAGLEATTEWLDSEDKILEKMPLLNRDQIKGWKAVFSEDGGWLAAAKAINAIGRFLRDQGVKFGFGGAGSFKQPLLAEGVCVGVETVDGTRYYADKVVLAAGAWSPALVDLQDQCVSKAWVYAHIQLSPSEAAEYKNVPVVYNGDVGFFFEPDEYGVIKVCDEFPGFTRFKQHQPFGASAPKRISVPRSAAKHPTDTYPDASEVSIRKAIATFLPKFTEKEVFNRHLCWCTDTADAALLMCEHPEWKNFVLATGDSGHTFKLLPNIGKHVVELLEGTLADDLAHAWRWRPGTGDALKSRRAARAKDLADMPGWNHDGEAPRAKL

SEQ ID NO: 122 - DNA, 1326 bp, Ulocladium sp.
atggcacctaacagagctaatatttctgtcatcgtcgtgggtggtggcggcaccattgggtcttcaacggcccttcatctcgtacgctcgggatacacaccgtcgaatatcacggttctggacacttatccaattccatcagcgcaatcagctggcaatgacttgaacaagatcatgggtatccgtttgcggaacaaggtggatttgcagttgagcttagaggcgagacaaatgtggacagaagacgatctgttcaaggagtactttcataaaaccgggcggctcgactgcgcacatggcgagaaaggccttgcagatctcaaacaagcctaccaagcccttcttgatgcgaacgctggcctggaggcgacgacagaatggttagattccgaggacaagattcttgagaagatgccgcttctcaatcgcgatcagatcaaaggatggaaagccgtcttcagcgaagacggcggatggctcgctgcggcaaaagccatcaacgctatcggtagatttctgcgcgatcaaggcgtcaagtttggctttggcggagcaggatcattcaaacaacctcttcttgccgagggtgtttgtgttggtgttgaaacagttgacgggacgagatattatgctgacaaggttgtgttggcggctggtgcgtggagtcctgcattggtcgatctacaagaccaatgtgtgtcgaaagcatgggtatacgctcacatccaactgtccccgagcgaggcggcggaatacaaaaatgttcctgtagtctataatggcgacgtgggcttcttcttcgagcctgacgaatacggcgtcatcaaagtctgtgacgagtttccaggttttacgcgcttcaagcagcatcaacctttcggcgcatcggctccaaagcgcatttctgtgcctcgatctgccgcaaaacaccccacagatacctatccggacgcctcggaagtcagtatccgcaaggccatcgcgacgttcctgcccaagttcacagaaaaggaagtgttcaacaggcatctgtgttggtgtactgatacggctgatgcggcgcttttgatgtgcgaacatcctgagtggaagaactttgttttggccacgggtgacagtggtcacaccttcaagcttctacctaacatcggtaagcatgtggtcgagctactagagggtacattagcagacgacctagcgcatgcgtggagatggcgtcccggtaccggcgatgcgctgaagtcgcgaagggcggcgcgtgcgaaagaccttgcagatatgccaggatggaatcatgacggggaagcccccagagcgaagctgtga

SEQ ID NO: 123 - protein, 437 aa, Penicillium janthinellum
MAHSRESTKIVIVGGGGTMGSSTALHLIRSGYTPSNITVLDVYPIPSLQSAGYDLNKIMSIRLRNGPDLQLSLEALDMWKNDPLFKPFFHNVGMLDCSSSQEGIASLRRKHQDLIDANIGLEKTNIWLESEDDILAKAPHFTREQIKGWKGLFCGDGGWLAAAKAINAIGTFLKSQGVKFGFGSAGTFKRPLFAPDGATCSGVETVDGTKYFADKVVLAAGAWSSTLVDLEDQCVSKAWVFAHIQLTPQESAQYKDVPVVYDGDYGFFFEPNEHGVIKVCDEFPGFSRFKLHQPYGATSPKLISVPRSHAKHPTDTYPDSSEETIRKAIARFMPRFKDKELFNRSMCWCTDTADANLLICEHPKWKNFILATGDSGHSFKVLPNIGKHVVELIEGRLPQDLAGAWRWRPGGDALKSKRSAPAKDLAEMPGWKHDAKL

SEQ ID NO: 124 - DNA, 1314 bp, Penicillium janthinellum
atggctcattcgcgagaaagcacaaagattgtcattgtcgggggaggtggcacaatgggatcttcaaccgcgctacacctgatacgctctggatacaccccgtcaaacatcaccgtccttgatgtatacccaattccatccttgcaatccgcaggatatgatcttaacaagatcatgagcatccgattacgcaacgggcctgacttgcaactttccctggaggctctcgatatgtggaaaaacgatccgttgttcaagcctttctttcacaacgttggcatgctagactgttcatcgtcacaagagggtattgcaagccttcgacggaagcaccaagacctcatagacgcgaatatcggactagagaagacgaatatctggttagagagtgaagatgatattctggcaaaagccccgcacttcacgcgggaacagatcaaggggtggaagggcttgttttgcggcgatggaggatggcttgctgcagccaaggccatcaatgcgatcggaacctttctaaaaagtcaaggcgtcaagttcggatttggaagtgccgggactttcaagcgacctttgtttgctccagatggggcgacatgcagcggtgttgagacagtagatggaacaaaatacttcgccgacaaggtggttttggccgctggtgcttggagttcgacgttagtagatttggaggaccaatgtgtttcgaaggcctgggtcttcgctcatatccaactcacgccccaagaatcggcccagtacaaggacgtgcccgtagtatacgacggtgattatggctttttcttcgagcccaacgaacacggagtaatcaaagtctgcgatgagttccccgggttctcccgcttcaagctgcatcaaccttacggtgccacctctcctaagcttatatccgttcctcgatcacacgccaagcatcccaccgatacctacccagattcttctgaagagaccattcgaaaagcgattgcgaggtttatgccacgcttcaaggataaggagctttttaataggagcatgtgctggtgcaccgatactgctgatgccaacttgttgatctgcgagcaccccaagtggaagaactttatcttggccacaggagacagcggccatagtttcaaggttttgcccaatataggaaaacatgtcgttgagttgatagaaggacgcctaccacaagacctggctggtgcgtggagatggagaccagggggagatgcccttaagtccaaacgcagtgctccggcaaaggaccttgctgaaatgccgggctggaagcatgatgcgaagctctga

SEQ ID NO: 125 - protein, 445 aa, Aspergillus fumigatus
MAPSILSTESSIIVIGAGTWGCSTALHLARRGYKDVTVLDPHPVPSPIAAGNDINKIMEHSELKDGSSDPRSAAFSTFTRAALKAWKTDPVFQPYFHETGFIISGHTPALIDHIRKDEVEPSETNFVKLETAEDFRRTMPPGVLTGDFPGWKGWLHKSGAGWIHAKKAMISAFNEAKRLGVRFVTGSPEGNVVSLVYEDGDVVGARTADGRVHKAHRTILSAGAGSDSLLDFKKQLRPTAWTLCHIQMGPEEVKQYRNLPVLFNIAKGFFMEPDEDKHELKICDEHPGYCNFLPDPNRPGQEKSVPFAKHQIPLEAEARARDFLHDTMPHLADRPLSFARICWDADTPDRAFLIDRHPEHPSLLVAVGGSGNGAMQMPTIGGFIADALESKLQKEVKDIVRWRPETAVDRDWRATQNRFGGPDRIMDFQQVGEDQWTKIGESRGP

SEQ ID NO: 126 - DNA, 1338 bp, Aspergillus fumigatus
atggcgccttcaattttgagcactgaatcttccattatcgttatcggagcaggcacatggggctgctcaactgctctgcacctcgctcgtcgaggctacaaagatgtcactgttctcgaccctcatccagttccttcgcccattgcagcaggcaatgacatcaacaagattatggagcacagcgagctgaaagatggctcatccgaccctcgaagcgcagccttctcgacatttacgcgagctgctcttaaggcgtggaaaactgacccggttttccagccttactttcacgaaactggctttatcatatcggggcacacacctgctctgattgaccacatacgaaaagacgaggtagaaccgtcagaaacaaacttcgtcaagctggagacagccgaggacttccgccggaccatgccgccaggtgtactgacaggcgacttccctggctggaaaggctggttgcacaagtctggtgctgggtggattcatgccaaaaaggctatgatctctgctttcaatgaagctaagcgcttgggagtcagatttgtcactggctctccggaagggaatgttgtatcgttggtatacgaggacggagacgtcgttggagccagaactgccgatggtcgcgtgcacaaagcccatcgcactattctttcggcaggtgctggcagtgacagtctcctagacttcaagaagcagcttcggcctaccgcgtggactctctgtcatattcagatgggccctgaagaggtcaagcaatatcggaaccttcctgtgttgttcaacatcgccaaagggttcttcatggagcctgatgaggataaacacgagctcaagatttgtgacgagcatccagggtactgcaactttctccctgacccaaacagaccgggccaggagaagagtgtccccttcgcaaagcatcagatcccgctcgaggccgaagcccgcgcacgagactttctccatgatacaatgccgcatctggctgaccggccactgtctttcgcgcgtatttgctgggatgctgataccccagaccgtgctttcttgatcgatagacatcctgaacacccctcactgctagtcgctgttggaggttccggcaatggcgccatgcaaatgcctacaattggcggttttatcgcagatgctctagagagtaaactacagaaggaggtgaaggacatcgttcgatggaggccagagacggctgtcgatcgagattggagagcgactcagaatcgctttggcgggcctgacaggatcatggattttcagcaggtcggagaggatcagtggaccaagattggagagagcagaggtccgtaa

SEQ ID NO: 127 - protein, 445 aa, Aspergillus oryzae
MTSSKLTPTSSILIVGAGTWGCSTALHLARRGYKNVTVLDPHPVPSPIAAGNDINKIMEHREVKASETDPWSIAFSTCTRAALKGWKNDPVFQPYFHETGAIVSGHTASLIKHIQEHEIDSSDAEFIKLNTAEDFRKTMPPGILTGNFPGWKGWLNKTGAGWIHAKKAMFSAYTEAKRLGVTFITGSPEGDVVSLIYENGDVVGARTADGTVHRADHTILSAGAGSDRLLDFKKQLRPTAWTLCHIRMTPDEAKKYRNLPVLFNVAKGFFMEPDEDNHELKICDEHPGYCNFVPDPKHGGEVRSIPFAKHQIPLEAEARARDFLRDTMPHLADRPLSFARICWDADTVDRAFLIDRHPEYRSLLLAVGGSGNGAMQMPTIGGFIADALEGNLQKELKHALRWRPEIAAQRDWKDTQNRFGGPNKVMDFQKVGENEWTKIGDKSRL

SEQ ID NO: 128 - DNA, 1338 bp, Aspergillus oryzae
atgacatcctccaagttgactcccacatcatctatcttaattgtcggtgcagggacctggggttgttctactgctttacatcttgcccgtcgaggatacaaaaatgtcacggtcctagatccgcacccggtcccttctcccattgcagctggcaatgacattaacaagattatggagcacagggaggtaaaagcctctgaaaccgatccttggagtatcgccttctcaacatgcacacgagctgcactgaaaggttggaaaaacgacccagtattccagccatacttccatgaaacgggggcaatagtttctggccacaccgcctctttgattaaacatatacaagaacacgaaatcgactcgtcagacgccgagttcataaaattgaacaccgcagaggatttccgcaaaactatgcccccgggaatcctcactggcaacttccccggctggaagggctggctgaacaagaccggcgccggatggatccacgccaagaaggccatgttctccgcatacaccgaagcaaagcgcctaggagtcactttcatcaccggctcccctgaaggagacgttgtatctctaatttacgagaatggagacgtagtcggagccagaacggccgacggcaccgtccaccgagcagaccataccattctttccgcaggggctggcagtgatcgtctcctggactttaagaaacagctccgtcctaccgcctggacgctctgccacatcagaatgacgcccgacgaggccaagaagtaccggaatcttcctgtgctgttcaacgtcgctaaggggttcttcatggaacctgatgaggataatcatgagcttaagatctgcgacgagcatcctggatattgcaacttcgtcccggacccgaagcacggcggtgaggtgcgcagtatcccatttgcaaagcatcagattcctcttgaagccgaggcccgtgcaagggacttcctccgtgatacgatgcctcatcttgctgatcgaccactgtcttttgctcgtatatgctgggatgctgatacagtggatcgcgccttcttgatcgataggcatcctgagtatcgctctttactgcttgctgtcggtggatctggtaatggagccatgcaaatgcctaccattggtgggttcatagcggatgctctggagggaaacctgcaaaaggaactgaagcatgcactacggtggaggcctgagattgccgcccaacgagactggaaggatacgcaaaatagattcggaggtccgaataaagtaatggatttccaaaaggttggagagaatgagtggaccaagattggcgataagagtcggctttaa

SEQ ID NO: 129 - protein, 438 aa, Aspergillus fumigatus
MAVTKSSSLLIVGAGTWGTSTALHLARRGYTNVTVLDPYPVPSAISAGNDVNKVISSGQYSNNKDEIEVNEILAEEAFNGWKNDPLFKPYYHDTGLLMSACSQEGLDRLGVRVRPGEDPNLVELTRPEQFRKLAPEGVLQGDFPGWKGYFARSGAGWAHARNALVAAAREAQRMGVKFVTGTPQGRVVTLIFENNDVKGAVTGDGKIWRAERTFLCAGASAGQFLDFKNQLRPTAWTLVHIALKPEERALYKNIPVIFNIERGFFFEPDEERGEIKICDEHPGYTNMVQSADGTMMSIPFEKTQIPKEAETRVRALLKETMPQLADRPFSFARICWCADTANREFLIDRHPQYHSLVLGCGASGRGFKYLPSIGNLIVDAMEGKVPQKIHELIKWNPDIAANRNWRDTLGRFGGPNRVMDFHDVKEWTNVQYRDISKL

SEQ ID NO: 130 - DNA, 1317 bp, Aspergillus fumigatus
atggcggtaaccaagtcatcttcccttttgatcgtgggggcaggcacctggggcacatcgactgctctccacctggcacgaagaggatacacaaatgtgacggttctagatccctaccccgttccctcagccatctcggctgggaatgatgtgaacaaggtcatctcctccggccaatatagcaacaacaaggacgaaattgaggtcaacgagattctggctgaagaagcgttcaatggctggaagaacgaccccttgttcaaaccatactatcacgatactggattgctcatgtccgcctgctcccaggaaggcttggaccgccttggagtccgtgtcaggcccggtgaggaccccaaccttgtggaactgacacggccggagcaattccgcaaattagctcctgagggtgttctacagggagatttccccggctggaagggctactttgcgcgttcaggagctggttgggcccatgctcgcaatgcactcgtggctgctgcaagggaggctcagagaatgggcgtgaagttcgtaactggcactcctcagggcagagtagtcactctaatatttgagaataacgatgtcaaaggtgccgttaccggagacggcaagatttggcgtgcagagcgcacattcctctgcgccggtgccagcgctggtcagttcctcgacttcaagaatcagttgcgtccaacggcatggacgctggttcatattgctctgaagcctgaggagcgggctctttacaagaatatcccagttatcttcaacattgagagggggttcttcttcgaaccagatgaggagcgcggtgagattaagatctgcgacgaacatccggggtataccaatatggtacagtctgccgacggcacgatgatgagcattccttttgaaaagactcagattcctaaagaagccgagacgagggttagagctctgcttaaagagacgatgccacagcttgcagaccgtccattcagtttcgccaggatttgctggtgcgccgacactgccaaccgggagttcttgatcgatcgccatcctcagtaccattcgcttgtgctgggctgcggcgcttccggcagaggattcaaatatctaccttcaattggcaatctcatcgttgatgctatggaaggcaaggtccctcaaaagatccacgaactgattaaatggaacccagatattgctgccaatcgcaactggagggatactttggggagattcgggggtcccaacagagtaatggacttccacgacgtcaaggagtggacaaatgtacaatatagagatatttccaagttataa

SEQ ID NO: 131 - protein, 437 aa, Aspergillus terreus
MPVTKSSSILIIGAGTWGCSTALHLARRGYTNVTVLDPYPVPSAISAGNDVNKIISSGQYSSKKDEVEVNEIIAEQAFNGWKNDPIFKPYYHDTGVVMSATTQEGLERLGVRVRPEDEPDVAELTRPEQFRQLAPGVLKGNFPGWRGYHIRSNAGWAHARNALVAAAREAQRLGVRFVAGSPQGRVITLIFENNDVKGAVTADGKIWRAEQTILCAGAAAGQFLDFKDQLRPTAWTLVHIQLKPEERAQYKNMPVVFNIEKGFFFEPDEERGEIKICDEHPGYTNMTTGADGRVRSIPFEKTQVPREAEMRVRKLLSETMPQLADRPFSFARICWCADTPNREFIIDRHPEYPSLVLGCGASGRGFKYLPSIGSIIADAMEDKTPAKIHKLIRWSPEIAINRNWGDRLGRFGGPNRVMDFNEVKEWTNVTQRDISKL

SEQ ID NO: 132 - DNA, 1314 bp, Aspergillus terreus
atgccagtcaccaagtcttcgtcgatattgatcatcggggcgggcacctggggttgctcaactgccctgcatcttgcccgcagaggatacaccaatgtcactgtccttgacccgtacccggttccatcagccatttcggccggcaacgacgtcaacaagatcatctcgtccggccagtacagcagcaagaaggacgaggtcgaagtcaatgagattatcgccgaacaggccttcaatggctggaaaaatgaccccatcttcaagccgtactaccacgacaccggcgtcgtgatgtccgccaccacacaggaaggattggagcgtctgggggtccgcgtgcgacctgaagatgaacccgatgtagccgaattgactcggccggagcagttccgccagctggcccccggcgtcttgaagggtaacttccccggttggagggggtaccacattcgctcaaacgcgggctgggcgcatgcgcgcaacgccctggtcgccgcggcgcgggaggcacagcgcctgggtgtgcgcttcgtcgcgggatcgccgcagggcagagtcatcacgttgatttttgagaacaacgatgtgaagggtgccgtcacggcggacggcaagatctggcgggccgagcagactatcctctgcgctggtgcggccgccggccagtttctggatttcaaggaccaactgcgtcccactgcgtggactctggtccacatccagttgaagccggaagagcgtgcccagtataaaaacatgccggtggtcttcaacatcgagaaggggttcttcttcgagccggatgaggagcgtggtgaaatcaagatctgcgacgaacaccccgggtacacgaatatgaccacgggggccgacggccgcgtgaggagcattcccttcgagaagacgcaggttcctcgagaagcggagatgcgcgtccgcaagcttctgtctgaaacgatgcctcagcttgcggaccggccgttcagtttcgcaaggatctgctggtgtgcggatacccccaatcgcgagtttatcattgaccgtcatcccgaatacccgtcgcttgttcttgggtgtggtgcttcaggacgaggcttcaaatatcttccctcgatcggaagcatcatcgcagacgccatggaggacaaaaccccggcaaaaatccacaagctgatccgctggagcccggaaatcgcgatcaaccgtaactggggggacagattaggtcgatttggagggcccaaccgggtcatggatttcaatgaagtgaaggagtggactaatgtcacccaaagggacatctcgaagttatag

SEQ ID NO: 133 - protein, 437 aa, Coniochaeta sp.
MTSNRADTRVIVVGGGGTIGSSTALHLVRSGYAPANITVLDTFEIPSAQSAGHDLNKIMGIDLRNKVDLQMSLEARQMWKEDELFQPFFHNTGRMDCEHTPEGIEKLKKLYQKLHDAGAGLEKTHAWLDNEDEILSKMPLLQRDQIQGWKAIWSQDGGWLAAAKAINAIGQFLKERGVKFGFGGAGSFKQPLFDDEGTTCIGVETADGTKYYADKVVLAAGAWSPTLVDLEDQCCSKAWVYAHIQLTPEEAAEYKGVPVVYNGEFGFFFEPDEFGVIKVCDEFPGFSRFKEHQPYGAPSPKRISVPRSHAKHPTDTYPDASEVSIKKAIATFLPRFQDKELFNRALCWCTDTADAALLMCEHPKWKNFILATGDSGHSFKILPNVGKYVVELIEGRLPEEMAYQWRWRPGGDALKSRRAAPPKDLADMPGWKHDPKL

SEQ ID NO: 134 - DNA, 1314 bp, Coniochaeta sp.
atgacgtcgaatcgtgcagatacaagggtgattgtcgtcggtggcggaggaacgattggttcctcgacagcgctgcatcttgtgaggagtggttatgctcccgcaaatatcacggtcttggacacatttgagattccatcggctcaatcagccggccatgatctcaacaagatcatgggaatagatctgcgcaacaaggtggacctgcaaatgagtctagaggctagacagatgtggaaggaggatgagttattccagcccttctttcacaataccggcagaatggactgcgaacacacgcctgagggtatcgagaaactgaaaaagctgtaccagaaactgcacgatgccggtgcgggtctggagaagactcatgcctggttggacaacgaggatgagatcttatccaagatgccgttgcttcaacgtgaccaaatacaaggatggaaagcaatatggagtcaagatggcggctggttagctgcggcaaaggccatcaatgcgatcggacagttcttgaaagaacgtggtgtaaagttcggattcggcggcgctggatccttcaagcaaccccttttcgacgatgaaggcacaacttgcattggcgttgagacggcagatggtaccaaatattacgctgacaaggtggtcttagcagctggcgcatggagcccaaccctggtggacctggaagatcaatgttgctcgaaggcttgggtgtatgctcatattcagttgacgcctgaagaggccgctgagtataagggtgtcccagttgtgtataatggcgaatttggcttcttctttgagcctgatgagtttggtgtaataaaggtgtgcgacgagttcccaggattctcgcgcttcaaggaacatcaaccctatggcgccccatctccgaaacggatatcagtaccacgatcgcacgccaagcatcccacagacacttatccagacgcatccgaagtcagcatcaaaaaagcaatcgcgacgtttctccctcgatttcaggacaaggagctcttcaatcgcgccttgtgctggtgtacagacactgcggacgctgctctcttgatgtgtgaacaccccaaatggaagaatttcattctagcgaccggcgacagcggacactcattcaaaatcttgcctaacgtcggaaaatacgtagtcgagttgatagagggccgcctgccggaggaaatggcttatcaatggaggtggcggccaggaggcgatgcactcaagtctagacgtgcggcaccgccaaaagatcttgcagacatgccaggatggaaacatgatccgaaattgtaa

SEQ ID NO: 135 - protein, 437 aa, Phaeosphaeria nodorum
MAPSRANTSVIVVGGGGTIGSSTALHLVRSGYTPSNVTVLDAYPIPSSQSAGNDLNKIMGVDLRNPVDLQLALEARQMWNEDELFKKFFHNTGRLDCAHGEKDIAKLKSLYQKLVDAGLDATNEWLDSEDEILKRMPLLSRDQIKGWKAIFSKDGGWLAAAKAINAVGEYLRDQGVRFGFYGAGSFKAPLLAEGVCIGVETVDGTRYYADKVVLAAGAWSPTLVELHEQCVSKAWVYGHIQLTPEEAARYKNSPVVYNGDVGFFFEPNEHGVIKVCDEFPGFTRFKMHQPFGAKAPKRISVPRSHAKHPTDTIPDASDVSIRRAIATFMPQFKNKKMFNQAMCWCTDTADAALLICEHPEWKNFVLATGDSGHSFKLLPNIGKHVVELLEGTLADDLAHAWRWRPGSGDALKSRRSAPAKDLADMPGWNHDKPRANL

SEQ ID NO: 136 - DNA, 1314 bp, Phaeosphaeria nodorum
atggccccgtcgcgtgctaatacgtcggtcattgtggttggtggtggtggtacgattggctcatctacggctctgcatctggtccgctcaggctataccccgtcgaacgtgacggttctggatgcatacccgattccgagctctcagagcgctggcaacgacctgaataaaatcatgggtgtcgatctgcgtaatccggtggatctgcagctggctctggaagcgcgccaaatgtggaacgaagacgaactgttcaagaagtttttccataacaccggccgtctggattgcgcgcacggtgaaaaagatattgccaaactgaagagcctgtatcagaaactggtggatgcgggtctggacgccacgaacgaatggctggatagtgaagacgaaatcctgaaacgtatgccgctgctgtcccgcgatcaaattaaaggctggaaggcgatcttttcaaaagacggtggttggctggcagcagcaaaggcaattaatgcagttggtgaatatctgcgtgatcagggcgtccgcttcggtttttacggcgccggttctttcaaagcaccgctgctggctgaaggcgtctgcatcggtgtcgaaaccgtggatggcacgcgctattacgcagacaaagtggttctggctgcaggtgcatggtcgccgaccctggttgaactgcatgaacagtgtgtgagcaaagcgtgggtttacggccacattcaactgacgccggaagaagccgcacgttataagaacagcccggtcgtgtacaatggcgatgtgggctttttctttgaaccgaacgaacatggcgttatcaaagtctgcgatgaatttccgggttttacccgcttcaagatgcaccagccgtttggtgccaaagcaccgaagcgtattagtgtgccgcgctcccatgccaaacacccgaccgatacgatcccggatgcaagtgacgtttccattcgtcgcgctatcgcgacctttatgccgcagttcaagaacaaaaagatgttcaaccaagcgatgtgctggtgtaccgatacggccgacgctgcgctgctgatttgtgaacatccggaatggaaaaactttgttctggcgaccggcgattcaggtcattcgttcaaactgctgccgaatatcggcaagcacgttgtcgaactgctggagggtacgctggcagatgacctggcacacgcatggcgttggcgtccgggtagtggtgatgcactgaaaagccgtcgctctgctccggcgaaagacctggctgatatgccgggctggaaccatgacaaaccgcgtgctaatctgtaa

SEQ ID NO: 137 - protein, 441 aa, Neocosmospora vasinfecta
MTTPRKETTVLIIGGGGTIGSSTALHLLRAGYTPSNITVLDTYPIPSAQSAGNDLNKIMGIDLRNKVDLQLSLEARDMWRNDALFRPFFHNTGRLDCESSAEGVEKLRRLYQKLVEAGVGLEETHEWLDSEEAILEKAPLLQREEIEGWKAIWSEEGGWLAAAKAINAIGEELQRQGVRFGFGGAGSFKRPLFADDGTTCIGVETVDGTQYHADKVVLAAGAWSPALVDLEEQCCSKAWVYAHMQLTPEEAAVYKGCPVVYHGDVGFFFEPNENGVIKVCDEFPGFTRFKQHQPYGAPAPKPVSVPRSHAKHPTDTYPDASEESIKRAVSTFLPRFKDKPLFNRALCWCTDTADSALLICEHPRWKNFILATGDSGHSFKLLPIIGKHVVELVEGRLADDLAEAWRWRPGQGDARKSIRAAPAKDLADMPGWKHDQDSESR

SEQ ID NO: 138 - DNA, 1326 bp, Neocosmospora vasinfecta
atgacgaccccgcgtaaagaaacgacggtcctgattattggtggtggtggcacgattggtagctcgacggctctgcatctgctgcgtgccggctataccccgtctaacattaccgtgctggatacgtacccgatcccgagtgcccagtccgcaggcaacgacctgaataaaattatgggtatcgatctgcgcaataaagttgatctgcaactgagcctggaagcccgtgatatgtggcgcaacgacgcactgtttcgtccgtttttccataataccggccgcctggactgcgaaagctctgctgaaggcgtggaaaaactgcgtcgcctgtatcagaaactggtggaagcaggcgttggtctggaagaaacgcacgaatggctggatagcgaagaagctattctggaaaaagcgccgctgctgcaacgtgaagaaattgaaggttggaaagccatctggtctgaagaaggcggttggctggcggccgcaaaagctattaacgcgatcggcgaagaactgcagcgtcaaggcgttcgcttcggttttggcggtgccggtagttttaaacgcccgctgttcgcagatgacggcaccacgtgtatcggtgtcgaaaccgtggatggcacgcagtatcatgcggacaaagtggttctggctgcaggtgcttggtcaccggcgctggtcgatctggaagaacagtgctgttcgaaagcctgggtgtacgcacacatgcaactgaccccggaagaagccgcagtttataaaggctgcccggtcgtgtaccacggcgatgtcggctttttctttgaaccgaacgaaaatggcgttattaaagtctgtgacgaattcccgggttttacgcgtttcaaacagcatcaaccgtatggtgccccggcaccgaaacctgtgagtgttccgcgctcccatgcgaaacacccgaccgatacgtacccggacgcttcagaagaatcgatcaaacgtgccgtgagtacctttctgccgcgcttcaaagataaaccgctgtttaaccgtgcactgtgctggtgtaccgatacggccgactccgcactgctgatttgcgaacacccgcgctggaaaaattttatcctggcgaccggcgatagcggtcattctttcaaactgctgccgattatcggcaaacacgttgtcgaactggttgaaggtcgtctggcggatgacctggctgaagcgtggcgttggcgtccgggtcagggtgatgcacgtaaaagcattcgcgctgcgccggcgaaagacctggcggatatgccgggctggaaacacgaccaagactcggaatcacgctga

SEQ ID NO: 139 - protein, 438 aa, Aspergillus nidulans
MTPRANTKIIVVGGGGTMGSSTALHLLRAGYTPSNITVLDTCPIPSAQSAGYDLNKIMGIDLRNKPDLQLSLEALDMWKNDPLFKPFFHNVGMIDVSSTEEGIEKLRKLYQSLLDAGIGLEKTNFMLESEDEILAKAPHFTQEQIKGWKGLFCGDGGWLAAAKAINAIGQFLKEQGVKFGFGGAGTFKKPLFADAHEKTCIGVETVDGTKYYADKVVLAAGAWSSTLVDLEEQCVSKAWVFAHIQLTPAEAAAYKNTPVIYDGDYGFFFEPNENGIIKVCDEFPGFTHFKMHQPYGSPAPKPISVPRSHAKHPTDTYPHASEVTIKKAINRFLPRFNDKELFNRAMCWCTDTADANLLVCEHPRWKGFYLATGDSGHSFKLLPNIGKHVVELLEERLESVFKDAWRWRPGSGDALKSRRAAPAKDLADMPGWRNEAKM

SEQ ID NO: 140 - DNA, 1317 bp, Aspergillus nidulans
atgacgccccgagccaacaccaaaatcattgtcgtcggcggcggcggcacaatgggctcgtcgacagccctacacctcctgcgcgccggctacacgccgtccaacattacagtgctcgacacgtgccctatcccctccgcacagtctgcaggctacgacctgaacaaaatcatgggcatcgatctgcgcaacaagcctgatttacagctctctcttgaggcgctggacatgtggaaaaatgatcctctcttcaagccgtttttccacaatgttggaatgatcgacgtctcttcaacagaggaaggcatcgagaaacttcggaagctgtaccagtctcttctcgacgcaggcattgggctcgagaagacgaatttcatgctggaaagtgaagacgagatcctggctaaagcgccgcatttcacgcaggagcagattaaaggctggaaaggcctgttctgtggcgacggcggctggctcgctgcagccaaagccatcaatgccattgggcagttcctcaaggaacagggcgtcaagtttggattcggcggcgccggcacgttcaaaaagccactcttcgccgatgcccacgagaagacgtgcatcggcgtcgagactgtagacggcacaaagtactacgccgacaaggtcgttctagcagctggtgcctggagttcgacgttggtcgatctggaggagcagtgcgtttcaaaggcctgggtctttgcccacatccaactgacgcccgctgaagcagccgcgtataagaacactcctgttatatacgacggtgactatgggtttttctttgagccgaatgaaaacggcatcataaaagtctgtgacgaattccctggcttcacgcatttcaaaatgcaccagccgtacggctcgccggcgcccaaacccatctctgtgcctcgttcccatgcgaagcaccccacagatacatacccgcacgcgtcggaggtcacgatcaaaaaggctatcaaccggttcctgccgaggttcaatgacaaggaactgtttaacagggccatgtgctggtgcaccgataccgcggatgcaaatctgcttgtttgtgagcatccacgctggaaggggttttatcttgcaacaggggacagtgggcattcgttcaagttgctgccgaatattggaaagcatgttgtcgagttattggaggagaggctggaaagtgtgtttaaggatgcttggaggtggaggcctggcagtggggatgcattaaaaagtagacgggctgcgcctgcgaaggacctggcggatatgccggggtggaggaatgaggcaaagatgtag

SEQ ID NO: 141 - protein, 437 aa, Coniochaeta sp.
MTSNRADTRVIVVGGGGTIGSSTALHLVRSGYAPANITVLDTFEIPSAQSAGHDLNKIMGIDHRNKVDLQMSLEARQMWKEDELFQPFFHNTGRMDCEHTPKGIEKLKKLYQKLHDAGAGLEKTHAWLDNEDEILSKMPLLQRDQIQGWKAIWSQDGGWLAAAKAINAIGQFLKERGVKFGFGGAGSFKQPLFDDEGTTCIGVETADGTKYYADKVVLAAGAWSPTLVDLEDQCCSKAWVYAHIQLTPEEAAEYKGVPVVYNGEFGFFFEPDEFGVIKVCDEFPGFSRFKEHQPYGAPSPKRISVPRSHAKHPTDTYPDASEVSIKKAIATFLPRFQDKELFNRALCWCTDTADSALLMCEHPKWKNFILATGDSGHSFKILPNVGKYVVELIEGRLPEEMAYQWRWRPGGDALKSRRAAPPKDLADMPGWKHDPKL

SEQ ID NO: 142 - DNA, 1314 bp, Coniochaeta sp.
atgacgtcgaatcgtgcagatacaagggtgattgtcgtcggtggcggaggaacgattggttcctcgacagcgctgcatcttgtgaggagtggttatgctcccgcaaatatcacggtcttggacacatttgagattccatcggctcaatcagccggccatgatctcaacaagatcatgggaatagatcatcgcaacaaggtggacctgcaaatgagtctagaggctagacagatgtggaaggaggatgagttattccagcccttctttcacaataccggcagaatggactgcgaacacacgcctaagggtatcgagaaactgaaaaagctgtaccagaaactgcacgatgccggtgcgggtctggagaagactcatgcctggttggacaacgaggatgagatcttatccaagatgccgttgcttcaacgtgaccaaatacaaggatggaaagcaatatggagtcaagatggcggctggttagctgcggcaaaggccatcaatgcgatcggacagttcttgaaagaacgtggtgtaaagttcggattcggcggcgctggatccttcaagcaaccccttttcgacgatgaaggcacaacttgcattggcgttgagacggcagatggtaccaaatattacgctgacaaggtggtcttagcagctggcgcatggagcccaaccctggtggacctggaagatcaatgttgctcgaaggcttgggtgtatgctcatattcagttgacgcctgaagaggccgctgagtataagggtgtcccagttgtgtataatggcgaatttggcttcttctttgagcctgatgagtttggtgtaataaaggtgtgcgacgagttcccaggattctcgcgcttcaaggaacatcaaccctatggcgccccatctccgaaacggatatcagtaccacgatcgcacgccaagcatcccacagacacttatccagacgcatccgaagtcagcatcaaaaaagcaatcgcgacgtttctccctcgatttcaggacaaggagctcttcaatcgcgccttgtgctggtgtacagacactgcggactctgctctcttgatgtgtgaacaccccaaatggaagaatttcattctagcgaccggcgacagcggacactcattcaaaatcttgcctaacgtcggaaaatacgtagtcgagttgatagagggccgcctgccggaggaaatggcttatcaatggaggtggcggccaggaggcgatgcactcaagtctagacgtgcggcaccgccaaaagatcttgcagacatgccaggatggaaacatgatccgaaattgtaa

SEQ ID NO: 143 - protein, 437 aa, Eupenicillium terrenum
MAHSRASTKVVVVGGGGTIGSSTALHLIRSGYTPSNITVLDVYKTPSLQSAGHDLNKIMGIDHRNGPDLQLSLESLDMWQNDELFKPFFHQVGMIDCSSSKEGIEKLRRLYQKLLDAGIGLEKTNVWLESEDEILAKAPNFTREQVKGWKGLFCTDGGWLAAAKAINAIGIFLQDKGVKFGFGDAGTFQQPLFAADGKTCIGLETTDGTKYFADKVVLAAGAWSPTLVDLEDQCVSKAWVFAHIQLTPKEADAYKNVPVVYDGEYGFFFEPDEYGVIKVCDEFPGFSRFKLHQPYGAASPKMISVPRSHAKHPTDTYPDASEVTIRKAIARFLPEFKDKELFNRTMCWCTDTADSNLLICEHPKWKNFILATGDSGHSFKLLPNIGKYVVELLEGSLSQEMAGAWRWRPGGDALRSRRGAPAKDLAEMPGWKHDAHL

SEQ ID NO: 144 - DNA, 1314 bp, Eupenicillium terrenum
atggctcattcgcgtgcaagcaccaaagtcgtcgtggttgggggaggtggtacgatcgggtcttcgacggctctgcacttaatccgctctggatataccccctcaaatatcaccgtgcttgacgtatacaagaccccttcattgcaatctgcaggacatgatttgaacaagatcatgggcattgatcatcgcaacgggcctgacttgcagctttcgctggaatcactcgacatgtggcaaaacgatgagttgttcaagccattctttcaccaagtgggcatgattgattgttcgtcatccaaagagggtattgaaaaacttcgacgattataccagaaactcctcgatgcgggcattgggctggagaagacgaacgtttggctggaatctgaagatgagatcctcgccaaagcgccgaatttcacgcgtgaacaagtcaaggggtggaaaggcttattttgcactgatggaggctggcttgctgcagccaaggctatcaatgcgatcggaattttcctccaggacaaaggtgtcaagtttggctttggagatgctggtacctttcagcaacctctgttcgccgctgatggaaaaacttgcatcggacttgaaactacagacggaaccaagtactttgctgacaaggttgtcttggctgctggtgcgtggagtcccaccttggtggatctagaagatcagtgtgtttcaaaggcctgggttttcgctcatattcaactcacacccaaagaagcggacgcgtacaagaatgtgcctgtggtctatgatggtgaatatgggttctttttcgaacccgacgagtatggggtgatcaaagtctgtgacgagttccctggtttctctcgcttcaaactgcatcaaccgtacggggctgcatctcccaagatgatatccgtaccgcgatcacacgccaagcatcccacagatacctaccctgatgcctccgaagtcaccatacgcaaagcgatcgcaaggttcctgccagaatttaaagacaaggagctcttcaaccgtaccatgtgctggtgtacagatacggccgattctaacttattgatttgcgaacacccgaagtggaagaatttcattctggccactggagatagcggacattccttcaagctgttgccaaacatcgggaaatacgtagttgagcttttagagggatctctatcgcaggaaatggctggtgcctggagatggagacccggaggtgatgctcttagatctagacgcggtgctccggcaaaggatcttgctgagatgccgggatggaagcatgatgcacatttgtga

SEQ ID NO: 145 - protein, 437 aa, Eupenicillium terrenum
MAHSRASTKVVVVGGGGTIGSSTALHLIRSGYTPSNITVLDVYKTPSLQSAGHDLNKIMGIRLRNGPDLQLSLESLDMWQNDELFKPFFHQVGMIDCSSSKEGIENLRRKYQTLLDAGIGLEKTNVWLESEDEILAKAPNFTREQVKGWKGLFCTDGGWLAAAKAINAIGIFLQDKGVKFGFGGAGTFQQPLFAADGKTCIGLETTDGTKYFADKVVLAAGAWSPTLVDLEDQCVSKAWVFAHIQLTPKEADAYKNVPVVYDGEYGFFFEPNEYGVIKVCDEFPGFSRFKLHQPYGAASPKMISVPRSHAKHPTDTYPDASEVTIRKAIARFLPEFKDKELFNRTMCWCTDTADANLLICEHPKWKNFILATGDSGHSFKLLPNIGKHVVELLEGSLSQEMAGAWRWRPGGDALRSRRGAPAKDLAEMPGWKHDAHL

SEQ ID NO: 146 - DNA, 1314 bp, Eupenicillium terrenum
atggctcattcgcgtgcaagcaccaaagtcgtcgtggttgggggaggtggtacgatcgggtcttcgacggctctgcacttaatccgctctggatataccccctcaaatatcaccgtgcttgacgtatacaagaccccttcattgcaatctgcaggacatgatttgaacaagatcatgggcattcgattgcgcaacgggcctgacttgcagctttcgctggaatcactcgacatgtggcaaaacgatgagttgttcaagccattctttcaccaagtgggcatgattgattgttcgtcatccaaagagggtattgaaaatcttcgacgaaaataccagaccctcctcgatgcgggcattgggctggagaagacgaacgtttggctggaatctgaagatgagatcctcgccaaagcgccgaatttcacgcgtgaacaagtcaaggggtggaaaggcttattttgcactgatggaggctggcttgctgcagccaaggctatcaatgcgatcggaattttcctccaggacaaaggtgtcaagtttggctttggaggtgctggaacatttcagcaacctctgttcgccgctgatggaaaaacttgcatcggacttgaaactacagacggaaccaagtactttgctgacaaggttgtcttggctgctggtgcgtggagtcccaccttggtggatctagaagatcagtgtgtttcaaaggcctgggttttcgctcatattcaactcacacccaaagaagcggacgcgtacaagaatgtgcctgtggtctatgatggtgaatatgggttcttttttgagcccaacgagtatggggtgatcaaagtctgtgacgagttccctggtttctctcgcttcaaactgcatcaaccgtacggggctgcatctcccaagatgatatccgtaccgcgatcacacgccaagcatcccacagatacctaccctgatgcctccgaagtcaccatacgcaaagcgatcgcaaggttcctgccagaatttaaagacaaggagctcttcaaccgtaccatgtgctggtgtacagatacggccgatgctaacttattgatttgcgaacacccgaagtggaagaatttcattctggccactggagatagcggacattccttcaagctgttgccaaacatcgggaaacacgttgttgagcttttagagggatctctatcgcaggaaatggctggtgcctggagatggagacccggaggtgatgctcttagatctagacgcggtgctccggcaaaggatcttgctgagatgccgggatggaagcatgatgcacatttgtga

SEQ ID NO: 147 - protein, 438 aa, Aspergillus nidulans
MTPRANTKIIVVGGGGTMGSSTALHLLRAGYTPSNITVLDTCPIPSAQSAGYDLNKIMSIRLRNKPDLQLSLEALDMWKNDPLFKPFFHNVGMIDVSSTEEGIEGLRKKYQSLLDAGIGLEKTNFMLESEDEILAKAPHFTQEQIKGWKGLFCGDGGWLAAAKAINAIGQFLKEQGVKFGFGGAGTFKKPLFADAHEKTCIGVETVDGTKYYADKVVLAAGAWSSTLVDLEEQCVSKAWVFAHIQLTPAEAAAYKNTPVIYDGDYGFFFEPNENGIIKVCDEFPGFTHFKMHQPYGSPAPKPISVPRSHAKHPTDTYPHASEVTIKKAINRFLPRFNDKELFNRAMCWCTDTADANLLVCEHPRWKGFYLATGDSGHSFKLLPNIGKHVVELLEERLESVFKDAWRWRPGSGDALKSRRAAPAKDLADMPGWRNEAKM

SEQ ID NO: 148 - DNA, 1317 bp, Aspergillus nidulans
atgacgccccgagccaacaccaaaatcattgtcgtcggcggcggcggcacaatgggctcgtcgacagccctacacctcctgcgcgccggctacacgccgtccaacattacagtgctcgacacgtgccctatcccctccgcacagtctgcaggctacgacctgaacaaaatcatgagcatcaggctgcgcaacaagcctgatttacagctctctcttgaggcgctggacatgtggaaaaatgatcctctcttcaagccgtttttccacaatgttggaatgatcgacgtctcttcaacagaggaaggcatcgagggtcttcggaagaaataccagtctcttctcgacgcaggcattgggctcgagaagacgaatttcatgctggaaagtgaagacgagatcctggctaaagcgccgcatttcacgcaggagcagattaaaggctggaaaggcctgttctgtggcgacggcggctggctcgctgcagccaaagccatcaatgccattgggcagttcctcaaggaacagggcgtcaagtttggattcggcggcgccggcacgttcaaaaagccactcttcgccgatgcccacgagaagacgtgcatcggcgtcgagactgtagacggcacaaagtactacgccgacaaggtcgttctagcagctggtgcctggagttcgacgttggtcgatctggaggagcagtgcgtttcaaaggcctgggtctttgcccacatccaactgacgcccgctgaagcagccgcgtataagaacactcctgttatatacgacggtgactatgggtttttctttgagccgaatgaaaacggcatcataaaagtctgtgacgaattccctggcttcacgcatttcaaaatgcaccagccgtacggctcgccggcgcccaaacccatctctgtgcctcgttcccatgcgaagcaccccacagatacatacccgcacgcgtcggaggtcacgatcaaaaaggctatcaaccggttcctgccgaggttcaatgacaaggaactgtttaacagggccatgtgctggtgcaccgataccgcggatgcaaatctgcttgtttgtgagcatccacgctggaaggggttttatcttgcaacaggggacagtgggcattcgttcaagttgctgccgaatattggaaagcatgttgtcgagttattggaggagaggctggaaagtgtgtttaaggatgcttggaggtggaggcctggcagtggggatgcattaaaaagtagacgggctgcgcctgcgaaggacctggcggatatgccggggtggaggaatgaggcaaagatgtag

SEQ ID NO: 149 - protein, 477 aa, Cryptococcus neoformans
MPPSRASTKVIVIGGGGTLGSSTALHLLRAGYTPSNITVLDTYLIPSAQSAGNDLNKIMGIRIRNPVDKQLSLEARDMWRNDEVFKPYFHNTGRLDCAHTPESIASLRKSYEAILKAGSGLEKTHHWLSTEDEILARAPLLDRKQIKGWKAIYSEDGGWLAAAKAINSIGQVLKEKGVTFGFGSAGSFKKPLFDEDGTKAIGIETVDGTQYFADKVVLAAGAWSPTLVDLEGQCCSKAWVYAHMQLTPEEAAEYKECPVVYNSELGFFFEPNEKGVIKVCDEFPGFTRFKQHQPYGASSTKHISFPRSHAKHPTDTIPDESDASIRRAISAFLPRFKEKELFNRALCWCTDTADANLLICEHPKWKNFILATGDSGHSFKILPNIGKHVVELIEGTLAEDLAESWRWRPGSGDPLISRRAAPARDLADLPGWNHDEPSDDDMDVKDVAVSLASVKIGENIGEKVVEDGARVGVKVLA

SEQ ID NO: 150 - DNA, 1434 bp, Cryptococcus neoformans
atgccaccttcgcgcgccagtactaaggtcatagttatcgggggcggtggtactctcgggtcctctactgctcttcaccttttacgagccggttacactccatccaacatcactgtgcttgacacgtatctaatcccatcagcacagtcggctggcaatgacctcaataagatcatgggtattcgtatcaggaatcctgtagataaacagttgagcctggaagcaagagacatgtggaggaatgatgaagttttcaagccttatttccacaacacgggaagacttgattgtgctcatacaccggagagcattgcatctttgcgtaaatcgtacgaggctatcttaaaggccgggagcgggctcgagaagacccaccattggctgagtacagaagatgaaatactggctagagcccctttgttggatcggaaacagatcaaaggatggaaagctatttacagcgaagatgggggctggcttgcggcggcgaaagctatcaacagtatcggccaggtgttgaaagagaaaggtgtgacattcggattcgggagtgcgggctcattcaagaaacccttgtttgacgaagacggtaccaaggccatcggcattgagacagttgatggtacgcaatattttgccgacaaggtcgttctggctgccggagcttggagtcctaccctcgtggatttggaagggcaatgctgttcaaaggcttgggtttacgcccatatgcaattgacaccagaagaggctgccgaatacaaggagtgtcctgtggtgtacaactctgaacttgggttcttcttcgagcccaatgaaaaaggagtcatcaaagtgtgcgacgaattcccagggttcacccgtttcaagcaacatcaaccttacggcgcctcctctactaaacacatctctttcccgcgctcccatgccaaacaccctaccgataccattccggacgagtcggacgcatctatccgccgtgctatctctgcctttttaccgagattcaaagaaaaagaactgttcaacagagcactgtgctggtgtacagataccgccgatgccaatcttttgatatgcgaacatcccaaatggaaaaattttatcttagctacaggggatagtggacattcattcaaaattcttcccaatatcggtaaacatgtcgttgaacttatagaaggtacccttgccgaggacttggctgagagctggagatggagacctggaagcggtgaccccctgatctctcgtcgggcagcccctgcaagggatcttgctgatcttccaggatggaaccatgatgagccctcggatgacgatatggatgtaaaggatgtcgctgtatcgcttgcttctgtgaaaattggcgaaaacatcggggagaaggttgtggaagatggagcacgagtcggagtcaaagttctagcttag

SEQ ID NO: 151 - protein, 437 aa, Coniochaeta sp.
MTSNRADTRVIVVGGGGTIGSSTALHLVRSGYAPANITVLDTFEIPSAQSAGHDLNKIMGIALRNKVDLQMSLEARQMWKEDELFQPFFHNTGRMDCEHTPEGIEDLKKQYQALHDAGAGLEKTHAWLDNEDEILSKMPLLQRDQIQGWKAIWSQDGGWLAAAKAINAIGQFLKERGVKFGFGGAGSFKQPLFDDEGTTCIGVETADGTKYYADKVVLAAGAWSPTLVDLEDQCCSKAWVYAHIQLTPEEAAEYKGVPVVYNGEFGFFFEPDEFGVIKVCDEFPGFSRFKEHQPYGAPSPKRISVPRSHAKHPTDTYPDASEVSIKKAIATFLPRFQDKELFNRALCWCTDTADAALLMCEHPKWKNFILATGDSGHSFKILPNVGKYVVELIEGRLPEEMAYQWRWRPGGDALKSRRAAPPKDLADMPGWKHDPKL

SEQ ID NO: 152 - DNA, 1314 bp, Coniochaeta sp.
atgacgtcgaatcgtgcagatacaagggtgattgtcgtcggtggcggaggaacgattggttcctcgacagcgctgcatcttgtgaggagtggttatgctcccgcaaatatcacggtcttggacacatttgagattccatcggctcaatcagccggccatgatctcaacaagatcatgggaatagcactgcgcaacaaggtggacctgcaaatgagtctagaggctagacagatgtggaaggaggatgagttattccagcccttctttcacaataccggcagaatggactgcgaacacacgcctgagggtatcgaggacctgaaaaagcagtaccaggcactgcacgatgccggtgcgggtctggagaagactcatgcctggttggacaacgaggatgagatcttatccaagatgccgttgcttcaacgtgaccaaatacaaggatggaaagcaatatggagtcaagatggcggctggttagctgcggcaaaggccatcaatgcgatcggacagttcttgaaagaacgtggtgtaaagttcggattcggcggcgctggatccttcaagcaaccccttttcgacgatgaaggcacaacttgcattggcgttgagacggcagatggtaccaaatattacgctgacaaggtggtcttagcagctggcgcatggagcccaaccctggtggacctggaagatcaatgttgctcgaaggcttgggtgtatgctcatattcagttgacgcctgaagaggccgctgagtataagggtgtcccagttgtgtataatggcgaatttggcttcttctttgagcctgatgagtttggtgtaataaaggtgtgcgacgagttcccaggattctcgcgcttcaaggaacatcaaccctatggcgccccatctccgaaacggatatcagtaccacgatcgcacgccaagcatcccacagacacttatccagacgcatccgaagtcagcatcaaaaaagcaatcgcgacgtttctccctcgatttcaggacaaggagctcttcaatcgcgccttgtgctggtgtacagacactgcggacgctgctctcttgatgtgtgaacaccccaaatggaagaatttcattctagcgaccggcgacagcggacactcattcaaaatcttgcctaacgtcggaaaatacgtagtcgagttgatagagggccgcctgccggaggaaatggcttatcaatggaggtggcggccaggaggcgatgcactcaagtctagacgtgcggcaccgccaaaagatcttgcagacatgccaggatggaaacatgatccgaaattgtaa

SEQ ID NO: 153 - protein, 437 aa, Coniochaeta sp.
MTSNRADTRVIVVGGGGTIGSSTALHLVRSGYAPANITVLDTFEIPSAQSAGHDLNKIMGIDLRNKVDLQMSLEARQMWKEDELFQPFFHNTGRMDCEHTPEGIEDLKKQYQALHDAGAGLEKTHAWLDNEDEILSKMPLLQRDQIQGWKAIWSQDGGWLAAAKAINAIGQFLKERGVKFGFGGAGSFKQPLFDDEGTTCIGVETADGTKYYADKVVLAAGAWSPTLVDLEDQCCSKAWVYAHIQLTPEEAAEYKGVPVVYNGEFGFFFEPDEFGVIKVCDEFPGFSRFKEHQPYGAPSPKRISVPRSHAKHPTDTYPDASEVSIKKAIATFLPRFQDKELFNRALCWCTDTADAALLMCEHPKWKNFILATGDSGHSFKILPNVGKYVVELIEGRLPEEMAYQWRWRPGGDALKSRRAAPPKDLADMPGWKHDPKL

SEQ ID NO: 154 - DNA, 1314 bp, Coniochaeta sp.
atgacgtcgaatcgtgcagatacaagggtgattgtcgtcggtggcggaggaacgattggttcctcgacagcgctgcatcttgtgaggagtggttatgctcccgcaaatatcacggtcttggacacatttgagattccatcggctcaatcagccggccatgatctcaacaagatcatgggaatagatctgcgcaacaaggtggacctgcaaatgagtctagaggctagacagatgtggaaggaggatgagttattccagcccttctttcacaataccggcagaatggactgcgaacacacgcctgagggtatcgaggacctgaaaaagcagtaccaggcactgcacgatgccggtgcgggtctggagaagactcatgcctggttggacaacgaggatgagatcttatccaagatgccgttgcttcaacgtgaccaaatacaaggatggaaagcaatatggagtcaagatggcggctggttagctgcggcaaaggccatcaatgcgatcggacagttcttgaaagaacgtggtgtaaagttcggattcggcggcgctggatccttcaagcaaccccttttcgacgatgaaggcacaacttgcattggcgttgagacggcagatggtaccaaatattacgctgacaaggtggtcttagcagctggcgcatggagcccaaccctggtggacctggaagatcaatgttgctcgaaggcttgggtgtatgctcatattcagttgacgcctgaagaggccgctgagtataagggtgtcccagttgtgtataatggcgaatttggcttcttctttgagcctgatgagtttggtgtaataaaggtgtgcgacgagttcccaggattctcgcgcttcaaggaacatcaaccctatggcgccccatctccgaaacggatatcagtaccacgatcgcacgccaagcatcccacagacacttatccagacgcatccgaagtcagcatcaaaaaagcaatcgcgacgtttctccctcgatttcaggacaaggagctcttcaatcgcgccttgtgctggtgtacagacactgcggacgctgctctcttgatgtgtgaacaccccaaatggaagaatttcattctagcgaccggcgacagcggacactcattcaaaatcttgcctaacgtcggaaaatacgtagtcgagttgatagagggccgcctgccggaggaaatggcttatcaatggaggtggcggccaggaggcgatgcactcaagtctagacgtgcggcaccgccaaaagatcttgcagacatgccaggatggaaacatgatccgaaattgtaa

SEQ ID NO: 155 - protein, 437 aa, Eupenicillium terrenum
MAHSRASTKVVVVGGGGTIGSSTALHLIRSGYTPSNITVLDVYKTPSLQSAGHDLNKIMGIDLRNGPDLQLSLESLDMWQNDELFKPFFHQVGMIDCSSSKEGIENLRRKYQTLLDAGIGLEKTNVWLESEDEILAKAPNFTREQVKGWKGLFCTDGGWLAAAKAINAIGIFLQDKGVKFGFGDAGTFQQPLFAADGKTCIGLETTDGTKYFADKVVLAAGAWSPTLVDLEDQCVSKAWVFAHIQLTPKEADAYKNVPVVYDGEYGFFFEPDEYGVIKVCDEFPGFSRFKLHQPYGAASPKMISVPRSHAKHPTDTYPDASEVTIRKAIARFLPEFKDKELFNRTMCWCTDTADANLLICEHPKWKNFILATGDSGHSFKLLPNIGKYVVELLEGSLSQEMAGAWRWRPGGDALRSRRGAPAKDLAEMPGWKHDAHL

SEQ ID NO: 156 - DNA, 1314 bp, Eupenicillium terrenum
atggctcattcgcgtgcaagcaccaaagtcgtcgtggttgggggaggtggtacgatcgggtcttcgacggctctgcacttaatccgctctggatataccccctcaaatatcaccgtgcttgacgtatacaagaccccttcattgcaatctgcaggacatgatttgaacaagatcatgggcattgatttgcgcaacgggcctgacttgcagctttcgctggaatcactcgacatgtggcaaaacgatgagttgttcaagccattctttcaccaagtgggcatgattgattgttcgtcatccaaagagggtattgaaaatcttcgacgaaaataccagaccctcctcgatgcgggcattgggctggagaagacgaacgtttggctggaatctgaagatgagatcctcgccaaagcgccgaatttcacgcgtgaacaagtcaaggggtggaaaggcttattttgcactgatggaggctggcttgctgcagccaaggctatcaatgcgatcggaattttcctccaggacaaaggtgtcaagtttggctttggagatgctggtacctttcagcaacctctgttcgccgctgatggaaaaacttgcatcggacttgaaactacagacggaaccaagtactttgctgacaaggttgtcttggctgctggtgcgtggagtcccaccttggtggatctagaagatcagtgtgtttcaaaggcctgggttttcgctcatattcaactcacacccaaagaagcggacgcgtacaagaatgtgcctgtggtctatgatggtgaatatgggttctttttcgaacccgacgagtatggggtgatcaaagtctgtgacgagttccctggtttctctcgcttcaaactgcatcaaccgtacggggctgcatctcccaagatgatatccgtaccgcgatcacacgccaagcatcccacagatacctaccctgatgcctccgaagtcaccatacgcaaagcgatcgcaaggttcctgccagaatttaaagacaaggagctcttcaaccgtaccatgtgctggtgtacagatacggccgatgctaacttattgatttgcgaacacccgaagtggaagaatttcattctggccactggagatagcggacattccttcaagctgttgccaaacatcgggaaatacgtagttgagcttttagagggatctctatcgcaggaaatggctggtgcctggagatggagacccggaggtgatgctcttagatctagacgcggtgctccggcaaaggatcttgctgagatgccgggatggaagcatgatgcacatttgtga

SEQ ID NO: 157 - protein, 437 aa, Coniochaeta sp.
MTSNRADTRVIVVGGGGTIGSSTALHLVRSGYAPANITVLDTFEIPSAQSAGHDLNKIMGIALRNKVDLQMSLEARQMWKEDELFQPFFHNTGRMDCEHTPEGIEDLKKLYQALHDAGAGLEKTHAWLDNEDEILSKMPLLQRDQIQGWKAIWSQDGGWLAAAKAINAIGQFLKERGVKFGFGGAGSFKQPLFDDEGTTCIGVETADGTKYYADKVVLAAGAWSPTLVDLEDQCCSKAWVYAHIQLTPEEAAEYKGVPVVYNGEFGFFFEPDEFGVIKVCDEFPGFSRFKEHQPYGAPSPKRISVPRSHAKHPTDTYPDASEVSIKKAIATFLPRFQDKELFNRALCWCTDTADAALLMCEHPKWKNFILATGDSGHSFKILPNVGKYVVELIEGRLPEEMAYQWRWRPGGDALKSRRAAPPKDLADMPGWKHDPKL

SEQ ID NO: 158 - DNA, 1314 bp, Coniochaeta sp.
atgacgtcgaatcgtgcagatacaagggtgattgtcgtcggtggcggaggaacgattggttcctcgacagcgctgcatcttgtgaggagtggttatgctcccgcaaatatcacggtcttggacacatttgagattccatcggctcaatcagccggccatgatctcaacaagatcatgggaatagcactgcgcaacaaggtggacctgcaaatgagtctagaggctagacagatgtggaaggaggatgagttattccagcccttctttcacaataccggcagaatggactgcgaacacacgcctgagggtatcgaggacctgaaaaagctgtaccaggcactgcacgatgccggtgcgggtctggagaagactcatgcctggttggacaacgaggatgagatcttatccaagatgccgttgcttcaacgtgaccaaatacaaggatggaaagcaatatggagtcaagatggcggctggttagctgcggcaaaggccatcaatgcgatcggacagttcttgaaagaacgtggtgtaaagttcggattcggcggcgctggatccttcaagcaaccccttttcgacgatgaaggcacaacttgcattggcgttgagacggcagatggtaccaaatattacgctgacaaggtggtcttagcagctggcgcatggagcccaaccctggtggacctggaagatcaatgttgctcgaaggcttgggtgtatgctcatattcagttgacgcctgaagaggccgctgagtataagggtgtcccagttgtgtataatggcgaatttggcttcttctttgagcctgatgagtttggtgtaataaaggtgtgcgacgagttcccaggattctcgcgcttcaaggaacatcaaccctatggcgccccatctccgaaacggatatcagtaccacgatcgcacgccaagcatcccacagacacttatccagacgcatccgaagtcagcatcaaaaaagcaatcgcgacgtttctccctcgatttcaggacaaggagctcttcaatcgcgccttgtgctggtgtacagacactgcggacgctgctctcttgatgtgtgaacaccccaaatggaagaatttcattctagcgaccggcgacagcggacactcattcaaaatcttgcctaacgtcggaaaatacgtagtcgagttgatagagggccgcctgccggaggaaatggcttatcaatggaggtggcggccaggaggcgatgcactcaagtctagacgtgcggcaccgccaaaagatcttgcagacatgccaggatggaaacatgatccgaaattgtaa

SEQ ID NO: 159 - protein, 437 aa, Coniochaeta sp.
MTSNRADTRVIVVGGGGTIGSSTALHLVRSGYAPANITVLDTFEIPSAQSAGHDLNKIMGIALRNKVDLQMSLEARQMWKEDELFQPFFHNTGRMDCEHTPEGIEDLKKYYQALHDAGAGLEKTHAWLDNEDEILSKMPLLQRDQIQGWKAIWSQDGGWLAAAKAINAIGQFLKERGVKFGFGGAGSFKQPLFDDEGTTCIGVETADGTKYYADKVVLAAGAWSPTLVDLEDQCCSKAWVYAHIQLTPEEAAEYKGVPVVYNGEFGFFFEPDEFGVIKVCDEFPGFSRFKEHQPYGAPSPKRISVPRSHAKHPTDTYPDASEVSIKKAIATFLPRFQDKELFNRALCWCTDTADAALLMCEHPKWKNFILATGDSGHSFKILPNVGKYVVELIEGRLPEEMAYQWRWRPGGDALKSRRAAPPKDLADMPGWKHDPKL

SEQ ID NO: 160 - DNA, 1314 bp, Coniochaeta sp.
atgacgtcgaatcgtgcagatacaagggtgattgtcgtcggtggcggaggaacgattggttcctcgacagcgctgcatcttgtgaggagtggttatgctcccgcaaatatcacggtcttggacacatttgagattccatcggctcaatcagccggccatgatctcaacaagatcatgggaatagcactgcgcaacaaggtggacctgcaaatgagtctagaggctagacagatgtggaaggaggatgagttattccagcccttctttcacaataccggcagaatggactgcgaacacacgcctgagggtatcgaggacctgaaaaagtattaccaggcactgcacgatgccggtgcgggtctggagaagactcatgcctggttggacaacgaggatgagatcttatccaagatgccgttgcttcaacgtgaccaaatacaaggatggaaagcaatatggagtcaagatggcggctggttagctgcggcaaaggccatcaatgcgatcggacagttcttgaaagaacgtggtgtaaagttcggattcggcggcgctggatccttcaagcaaccccttttcgacgatgaaggcacaacttgcattggcgttgagacggcagatggtaccaaatattacgctgacaaggtggtcttagcagctggcgcatggagcccaaccctggtggacctggaagatcaatgttgctcgaaggcttgggtgtatgctcatattcagttgacgcctgaagaggccgctgagtataagggtgtcccagttgtgtataatggcgaatttggcttcttctttgagcctgatgagtttggtgtaataaaggtgtgcgacgagttcccaggattctcgcgcttcaaggaacatcaaccctatggcgccccatctccgaaacggatatcagtaccacgatcgcacgccaagcatcccacagacacttatccagacgcatccgaagtcagcatcaaaaaagcaatcgcgacgtttctccctcgatttcaggacaaggagctcttcaatcgcgccttgtgctggtgtacagacactgcggacgctgctctcttgatgtgtgaacaccccaaatggaagaatttcattctagcgaccggcgacagcggacactcattcaaaatcttgcctaacgtcggaaaatacgtagtcgagttgatagagggccgcctgccggaggaaatggcttatcaatggaggtggcggccaggaggcgatgcactcaagtctagacgtgcggcaccgccaaaagatcttgcagacatgccaggatggaaacatgatccgaaattgtaa

SEQ ID NO: 161 - protein, 437 aa, Coniochaeta sp.
MTSNRADTRVIVVGGGGTIGSSTALHLVRSGYAPANITVLDTFEIPSAQSAGHDLNKIMGINLRNKVDLQMSLEARQMWKEDELFQPFFHNTGRMDCEHTPEGIEDLKKLYQALHDAGAGLEKTHAWLDNEDEILSKMPLLQRDQIQGWKAIWSQDGGWLAAAKAINAIGQFLKERGVKFGFGGAGSFKQPLFDDEGTTCIGVETADGTKYYADKVVLAAGAWSPTLVDLEDQCCSKAWVYAHIQLTPEEAAEYKGVPVVYNGEFGFFFEPDEFGVIKVCDEFPGFSRFKEHQPYGAPSPKRISVPRSHAKHPTDTYPDASEVSIKKAIATFLPRFQDKELFNRALCWCTDTADAALLMCEHPKWKNFILATGDSGHSFKILPNVGKYVVELIEGRLPEEMAYQWRWRPGGDALKSRRAAPPKDLADMPGWKHDPKL

SEQ ID NO: 162 - DNA, 1314 bp, Coniochaeta sp.
atgacgtcgaatcgtgcagatacaagggtgattgtcgtcggtggcggaggaacgattggttcctcgacagcgctgcatcttgtgaggagtggttatgctcccgcaaatatcacggtcttggacacatttgagattccatcggctcaatcagccggccatgatctcaacaagatcatgggaataaacctgcgcaacaaggtggacctgcaaatgagtctagaggctagacagatgtggaaggaggatgagttattccagcccttctttcacaataccggcagaatggactgcgaacacacgcctgagggtatcgaggacctgaaaaagctgtaccaggcactgcacgatgccggtgcgggtctggagaagactcatgcctggttggacaacgaggatgagatcttatccaagatgccgttgcttcaacgtgaccaaatacaaggatggaaagcaatatggagtcaagatggcggctggttagctgcggcaaaggccatcaatgcgatcggacagttcttgaaagaacgtggtgtaaagttcggattcggcggcgctggatccttcaagcaaccccttttcgacgatgaaggcacaacttgcattggcgttgagacggcagatggtaccaaatattacgctgacaaggtggtcttagcagctggcgcatggagcccaaccctggtggacctggaagatcaatgttgctcgaaggcttgggtgtatgctcatattcagttgacgcctgaagaggccgctgagtataagggtgtcccagttgtgtataatggcgaatttggcttcttctttgagcctgatgagtttggtgtaataaaggtgtgcgacgagttcccaggattctcgcgcttcaaggaacatcaaccctatggcgccccatctccgaaacggatatcagtaccacgatcgcacgccaagcatcccacagacacttatccagacgcatccgaagtcagcatcaaaaaagcaatcgcgacgtttctccctcgatttcaggacaaggagctcttcaatcgcgccttgtgctggtgtacagacactgcggacgctgctctcttgatgtgtgaacaccccaaatggaagaatttcattctagcgaccggcgacagcggacactcattcaaaatcttgcctaacgtcggaaaatacgtagtcgagttgatagagggccgcctgccggaggaaatggcttatcaatggaggtggcggccaggaggcgatgcactcaagtctagacgtgcggcaccgccaaaagatcttgcagacatgccaggatggaaacatgatccgaaattgtaa

SEQ ID NO: 163 - protein, 437 aa, Coniochaeta sp.
MTSNRADTRVIVVGGGGTIGSSTALHLVRSGYAPANITVLDTFEIPSAQSAGHDLNKIMGIDLRNKVDLQMSLEARQMWKEDELFQPFFHNTGRMDCEHTPEGIEDLKKLYQALHDAGAGLEKTHAWLDNEDEILSKMPLLQRDQIQGWKAIWSQDGGWLAAAKAINAIGQFLKERGVKFGFGGAGSFKQPLFDDEGTTCIGVETADGTKYYADKVVLAAGAWSPTLVDLEDQCCSKAWVYAHIQLTPEEAAEYKGVPVVYNGEFGFFFEPDEFGVIKVCDEFPGFSRFKEHQPYGAPSPKRISVPRSHAKHPTDTYPDASEVSIKKAIATFLPRFQDKELFNRALCWCTDTADAALLMCEHPKWKNFILATGDSGHSFKILPNVGKYVVELIEGRLPEEMAYQWRWRPGGDALKSRRAAPPKDLADMPGWKHDPKL

SEQ ID NO: 164 - DNA, 1314 bp, Coniochaeta sp.
atgacgtcgaatcgtgcagatacaagggtgattgtcgtcggtggcggaggaacgattggttcctcgacagcgctgcatcttgtgaggagtggttatgctcccgcaaatatcacggtcttggacacatttgagattccatcggctcaatcagccggccatgatctcaacaagatcatgggaatagatctgcgcaacaaggtggacctgcaaatgagtctagaggctagacagatgtggaaggaggatgagttattccagcccttctttcacaataccggcagaatggactgcgaacacacgcctgagggtatcgaggacctgaaaaagctgtaccaggcactgcacgatgccggtgcgggtctggagaagactcatgcctggttggacaacgaggatgagatcttatccaagatgccgttgcttcaacgtgaccaaatacaaggatggaaagcaatatggagtcaagatggcggctggttagctgcggcaaaggccatcaatgcgatcggacagttcttgaaagaacgtggtgtaaagttcggattcggcggcgctggatccttcaagcaaccccttttcgacgatgaaggcacaacttgcattggcgttgagacggcagatggtaccaaatattacgctgacaaggtggtcttagcagctggcgcatggagcccaaccctggtggacctggaagatcaatgttgctcgaaggcttgggtgtatgctcatattcagttgacgcctgaagaggccgctgagtataagggtgtcccagttgtgtataatggcgaatttggcttcttctttgagcctgatgagtttggtgtaataaaggtgtgcgacgagttcccaggattctcgcgcttcaaggaacatcaaccctatggcgccccatctccgaaacggatatcagtaccacgatcgcacgccaagcatcccacagacacttatccagacgcatccgaagtcagcatcaaaaaagcaatcgcgacgtttctccctcgatttcaggacaaggagctcttcaatcgcgccttgtgctggtgtacagacactgcggacgctgctctcttgatgtgtgaacaccccaaatggaagaatttcattctagcgaccggcgacagcggacactcattcaaaatcttgcctaacgtcggaaaatacgtagtcgagttgatagagggccgcctgccggaggaaatggcttatcaatggaggtggcggccaggaggcgatgcactcaagtctagacgtgcggcaccgccaaaagatcttgcagacatgccaggatggaaacatgatccgaaattgtaa

SEQ ID NO: 165 - protein, 437 aa, Coniochaeta sp.
MTSNRADTRVIVVGGGGTIGSSTALHLVRSGYAPANITVLDTFEIPSAQSAGHDLNKIMGIDLRNKVDLQMSLEARQMWKEDELFQPFFHNTGRMDCEHTPEGIEALKKLYQALHDAGAGLEKTHAWLDNEDEILSKMPLLQRDQIQGWKAIWSQDGGWLAAAKAINAIGQFLKERGVKFGFGGAGSFKQPLFDDEGTTCIGVETADGTKYYADKVVLAAGAWSPTLVDLEDQCCSKAWVYAHIQLTPEEAAEYKGVPVVYNGEFGFFFEPDEFGVIKVCDEFPGFSRFKEHQPYGAPSPKRISVPRSHAKHPTDTYPDASEVSIKKAIATFLPRFQDKELFNRALCWCTDTADAALLMCEHPKWKNFILATGDSGHSFKILPNVGKYVVELIEGRLPEEMAYQWRWRPGGDALKSRRAAPPKDLADMPGWKHDPKL

SEQ ID NO: 166 - DNA, 1314 bp, Coniochaeta sp.
atgacgtcgaatcgtgcagatacaagggtgattgtcgtcggtggcggaggaacgattggttcctcgacagcgctgcatcttgtgaggagtggttatgctcccgcaaatatcacggtcttggacacatttgagattccatcggctcaatcagccggccatgatctcaacaagatcatgggaatagatctgcgcaacaaggtggacctgcaaatgagtctagaggctagacagatgtggaaggaggatgagttattccagcccttctttcacaataccggcagaatggactgcgaacacacgcctgagggtatcgaggccctgaaaaagctgtaccaggcactgcacgatgccggtgcgggtctggagaagactcatgcctggttggacaacgaggatgagatcttatccaagatgccgttgcttcaacgtgaccaaatacaaggatggaaagcaatatggagtcaagatggcggctggttagctgcggcaaaggccatcaatgcgatcggacagttcttgaaagaacgtggtgtaaagttcggattcggcggcgctggatccttcaagcaaccccttttcgacgatgaaggcacaacttgcattggcgttgagacggcagatggtaccaaatattacgctgacaaggtggtcttagcagctggcgcatggagcccaaccctggtggacctggaagatcaatgttgctcgaaggcttgggtgtatgctcatattcagttgacgcctgaagaggccgctgagtataagggtgtcccagttgtgtataatggcgaatttggcttcttctttgagcctgatgagtttggtgtaataaaggtgtgcgacgagttcccaggattctcgcgcttcaaggaacatcaaccctatggcgccccatctccgaaacggatatcagtaccacgatcgcacgccaagcatcccacagacacttatccagacgcatccgaagtcagcatcaaaaaagcaatcgcgacgtttctccctcgatttcaggacaaggagctcttcaatcgcgccttgtgctggtgtacagacactgcggacgctgctctcttgatgtgtgaacaccccaaatggaagaatttcattctagcgaccggcgacagcggacactcattcaaaatcttgcctaacgtcggaaaatacgtagtcgagttgatagagggccgcctgccggaggaaatggcttatcaatggaggtggcggccaggaggcgatgcactcaagtctagacgtgcggcaccgccaaaagatcttgcagacatgccaggatggaaacatgatccgaaattgtaa

SEQ ID NO: 167 - protein, 437 aa, Coniochaeta sp.
MTSNRADTRVIVVGGGGTIGSSTALHLVRSGYAPANITVLDTFEIPSAQSAGHDLNKIMGIDLRNKVDLQMSLEARQMWKEDELFQPFFHNTGRMDCEHTPEGIEKLKKLYQALHDAGAGLEKTHAWLDNEDEILSKMPLLQRDQIQGWKAIWSQDGGWLAAAKAINAIGQFLKERGVKFGFGGAGSFKQPLFDDEGTTCIGVETADGTKYYADKVVLAAGAWSPTLVDLEDQCCSKAWVYAHIQLTPEEAAEYKGVPVVYNGEFGFFFEPDEFGVIKVCDEFPGFSRFKEHQPYGAPSPKRISVPRSHAKHPTDTYPDASEVSIKKAIATFLPRFQDKELFNRALCWCTDTADAALLMCEHPKWKNFILATGDSGHSFKILPNVGKYVVELIEGRLPEEMAYQWRWRPGGDALKSRRAAPPKDLADMPGWKHDPKL

SEQ ID NO: 168 - DNA, 1314 bp, Coniochaeta sp.
atgacgtcgaatcgtgcagatacaagggtgattgtcgtcggtggcggaggaacgattggttcctcgacagcgctgcatcttgtgaggagtggttatgctcccgcaaatatcacggtcttggacacatttgagattccatcggctcaatcagccggccatgatctcaacaagatcatgggaatagatctgcgcaacaaggtggacctgcaaatgagtctagaggctagacagatgtggaaggaggatgagttattccagcccttctttcacaataccggcagaatggactgcgaacacacgcctgagggtatcgagaaactgaaaaagctgtaccaggcactgcacgatgccggtgcgggtctggagaagactcatgcctggttggacaacgaggatgagatcttatccaagatgccgttgcttcaacgtgaccaaatacaaggatggaaagcaatatggagtcaagatggcggctggttagctgcggcaaaggccatcaatgcgatcggacagttcttgaaagaacgtggtgtaaagttcggattcggcggcgctggatccttcaagcaaccccttttcgacgatgaaggcacaacttgcattggcgttgagacggcagatggtaccaaatattacgctgacaaggtggtcttagcagctggcgcatggagcccaaccctggtggacctggaagatcaatgttgctcgaaggcttgggtgtatgctcatattcagttgacgcctgaagaggccgctgagtataagggtgtcccagttgtgtataatggcgaatttggcttcttctttgagcctgatgagtttggtgtaataaaggtgtgcgacgagttcccaggattctcgcgcttcaaggaacatcaaccctatggcgccccatctccgaaacggatatcagtaccacgatcgcacgccaagcatcccacagacacttatccagacgcatccgaagtcagcatcaaaaaagcaatcgcgacgtttctccctcgatttcaggacaaggagctcttcaatcgcgccttgtgctggtgtacagacactgcggacgctgctctcttgatgtgtgaacaccccaaatggaagaatttcattctagcgaccggcgacagcggacactcattcaaaatcttgcctaacgtcggaaaatacgtagtcgagttgatagagggccgcctgccggaggaaatggcttatcaatggaggtggcggccaggaggcgatgcactcaagtctagacgtgcggcaccgccaaaagatcttgcagacatgccaggatggaaacatgatccgaaattgtaa

SEQ ID NO: 169 - protein, 437 aa, Coniochaeta sp.
MTSNRADTRVIVVGGGGTIGSSTALHLVRSGYAPANITVLDTFEIPSAQSAGHDLNKIMGIDLRNKVDLQMSLEARQMWKEDELFQPFFHNTGRMDCEHTPEGIERLKKLYQALHDAGAGLEKTHAWLDNEDEILSKMPLLQRDQIQGWKAIWSQDGGWLAAAKAINAIGQFLKERGVKFGFGGAGSFKQPLFDDEGTTCIGVETADGTKYYADKVVLAAGAWSPTLVDLEDQCCSKAWVYAHIQLTPEEAAEYKGVPVVYNGEFGFFFEPDEFGVIKVCDEFPGFSRFKEHQPYGAPSPKRISVPRSHAKHPTDTYPDASEVSIKKAIATFLPRFQDKELFNRALCWCTDTADAALLMCEHPKWKNFILATGDSGHSFKILPNVGKYVVELIEGRLPEEMAYQWRWRPGGDALKSRRAAPPKDLADMPGWKHDPKL

SEQ ID NO: 170 - DNA, 1314 bp, Coniochaeta sp.
atgacgtcgaatcgtgcagatacaagggtgattgtcgtcggtggcggaggaacgattggttcctcgacagcgctgcatcttgtgaggagtggttatgctcccgcaaatatcacggtcttggacacatttgagattccatcggctcaatcagccggccatgatctcaacaagatcatgggaatagatctgcgcaacaaggtggacctgcaaatgagtctagaggctagacagatgtggaaggaggatgagttattccagcccttctttcacaataccggcagaatggactgcgaacacacgcctgagggtatcgagcgcctgaaaaagctgtaccaggcactgcacgatgccggtgcgggtctggagaagactcatgcctggttggacaacgaggatgagatcttatccaagatgccgttgcttcaacgtgaccaaatacaaggatggaaagcaatatggagtcaagatggcggctggttagctgcggcaaaggccatcaatgcgatcggacagttcttgaaagaacgtggtgtaaagttcggattcggcggcgctggatccttcaagcaaccccttttcgacgatgaaggcacaacttgcattggcgttgagacggcagatggtaccaaatattacgctgacaaggtggtcttagcagctggcgcatggagcccaaccctggtggacctggaagatcaatgttgctcgaaggcttgggtgtatgctcatattcagttgacgcctgaagaggccgctgagtataagggtgtcccagttgtgtataatggcgaatttggcttcttctttgagcctgatgagtttggtgtaataaaggtgtgcgacgagttcccaggattctcgcgcttcaaggaacatcaaccctatggcgccccatctccgaaacggatatcagtaccacgatcgcacgccaagcatcccacagacacttatccagacgcatccgaagtcagcatcaaaaaagcaatcgcgacgtttctccctcgatttcaggacaaggagctcttcaatcgcgccttgtgctggtgtacagacactgcggacgctgctctcttgatgtgtgaacaccccaaatggaagaatttcattctagcgaccggcgacagcggacactcattcaaaatcttgcctaacgtcggaaaatacgtagtcgagttgatagagggccgcctgccggaggaaatggcttatcaatggaggtggcggccaggaggcgatgcactcaagtctagacgtgcggcaccgccaaaagatcttgcagacatgccaggatggaaacatgatccgaaattgtaa

SEQ ID NO: 171 - protein, 437 aa, Coniochaeta sp.
MTSNRADTRVIVVGGGGTIGSSTALHLVRSGYAPANITVLDTFEIPSAQSAGHDLNKIMGIDLRNKVDLQMSLEARQMWKEDELFQPFFHNTGRMDCEHTPEGIEDLKKLYQKLHDAGAGLEKTHAWLDNEDEILSKMPLLQRDQIQGWKAIWSQDGGWLAAAKAINAIGQFLKERGVKFGFGGAGSFKQPLFDDEGTTCIGVETADGTKYYADKVVLAAGAWSPTLVDLEDQCCSKAWVYAHIQLTPEEAAEYKGVPVVYNGEFGFFFEPDEFGVIKVCDEFPGFSRFKEHQPYGAPSPKRISVPRSHAKHPTDTYPDASEVSIKKAIATFLPRFQDKELFNRALCWCTDTADAALLMCEHPKWKNFILATGDSGHSFKILPNVGKYVVELIEGRLPEEMAYQWRWRPGGDALKSRRAAPPKDLADMPGWKHDPKL

SEQ ID NO: 172 - DNA, 1314 bp, Coniochaeta sp.
atgacgtcgaatcgtgcagatacaagggtgattgtcgtcggtggcggaggaacgattggttcctcgacagcgctgcatcttgtgaggagtggttatgctcccgcaaatatcacggtcttggacacatttgagattccatcggctcaatcagccggccatgatctcaacaagatcatgggaatagatctgcgcaacaaggtggacctgcaaatgagtctagaggctagacagatgtggaaggaggatgagttattccagcccttctttcacaataccggcagaatggactgcgaacacacgcctgagggtatcgaggacctgaaaaagctgtaccagaaactgcacgatgccggtgcgggtctggagaagactcatgcctggttggacaacgaggatgagatcttatccaagatgccgttgcttcaacgtgaccaaatacaaggatggaaagcaatatggagtcaagatggcggctggttagctgcggcaaaggccatcaatgcgatcggacagttcttgaaagaacgtggtgtaaagttcggattcggcggcgctggatccttcaagcaaccccttttcgacgatgaaggcacaacttgcattggcgttgagacggcagatggtaccaaatattacgctgacaaggtggtcttagcagctggcgcatggagcccaaccctggtggacctggaagatcaatgttgctcgaaggcttgggtgtatgctcatattcagttgacgcctgaagaggccgctgagtataagggtgtcccagttgtgtataatggcgaatttggcttcttctttgagcctgatgagtttggtgtaataaaggtgtgcgacgagttcccaggattctcgcgcttcaaggaacatcaaccctatggcgccccatctccgaaacggatatcagtaccacgatcgcacgccaagcatcccacagacacttatccagacgcatccgaagtcagcatcaaaaaagcaatcgcgacgtttctccctcgatttcaggacaaggagctcttcaatcgcgccttgtgctggtgtacagacactgcggacgctgctctcttgatgtgtgaacaccccaaatggaagaatttcattctagcgaccggcgacagcggacactcattcaaaatcttgcctaacgtcggaaaatacgtagtcgagttgatagagggccgcctgccggaggaaatggcttatcaatggaggtggcggccaggaggcgatgcactcaagtctagacgtgcggcaccgccaaaagatcttgcagacatgccaggatggaaacatgatccgaaattgtaa

SEQ ID NO: 173 - protein, 437 aa, Coniochaeta sp.
MTSNRADTRVIVVGGGGTIGSSTALHLVRSGYAPANITVLDTFEIPSAQSAGHDLNKIMGIDLRNKVDLQMSLEARQMWKEDELFQPFFHNTGRMDCEHTPEGIEDLKKLYQRLHDAGAGLEKTHAWLDNEDEILSKMPLLQRDQIQGWKAIWSQDGGWLAAAKAINAIGQFLKERGVKFGFGGAGSFKQPLFDDEGTTCIGVETADGTKYYADKVVLAAGAWSPTLVDLEDQCCSKAWVYAHIQLTPEEAAEYKGVPVVYNGEFGFFFEPDEFGVIKVCDEFPGFSRFKEHQPYGAPSPKRISVPRSHAKHPTDTYPDASEVSIKKAIATFLPRFQDKELFNRALCWCTDTADAALLMCEHPKWKNFILATGDSGHSFKILPNVGKYVVELIEGRLPEEMAYQWRWRPGGDALKSRRAAPPKDLADMPGWKHDPKL

SEQ ID NO: 174 - DNA, 1314 bp, Coniochaeta sp.
atgacgtcgaatcgtgcagatacaagggtgattgtcgtcggtggcggaggaacgattggttcctcgacagcgctgcatcttgtgaggagtggttatgctcccgcaaatatcacggtcttggacacatttgagattccatcggctcaatcagccggccatgatctcaacaagatcatgggaatagatctgcgcaacaaggtggacctgcaaatgagtctagaggctagacagatgtggaaggaggatgagttattccagcccttctttcacaataccggcagaatggactgcgaacacacgcctgagggtatcgaggacctgaaaaagctgtaccagcgtctgcacgatgccggtgcgggtctggagaagactcatgcctggttggacaacgaggatgagatcttatccaagatgccgttgcttcaacgtgaccaaatacaaggatggaaagcaatatggagtcaagatggcggctggttagctgcggcaaaggccatcaatgcgatcggacagttcttgaaagaacgtggtgtaaagttcggattcggcggcgctggatccttcaagcaaccccttttcgacgatgaaggcacaacttgcattggcgttgagacggcagatggtaccaaatattacgctgacaaggtggtcttagcagctggcgcatggagcccaaccctggtggacctggaagatcaatgttgctcgaaggcttgggtgtatgctcatattcagttgacgcctgaagaggccgctgagtataagggtgtcccagttgtgtataatggcgaatttggcttcttctttgagcctgatgagtttggtgtaataaaggtgtgcgacgagttcccaggattctcgcgcttcaaggaacatcaaccctatggcgccccatctccgaaacggatatcagtaccacgatcgcacgccaagcatcccacagacacttatccagacgcatccgaagtcagcatcaaaaaagcaatcgcgacgtttctccctcgatttcaggacaaggagctcttcaatcgcgccttgtgctggtgtacagacactgcggacgctgctctcttgatgtgtgaacaccccaaatggaagaatttcattctagcgaccggcgacagcggacactcattcaaaatcttgcctaacgtcggaaaatacgtagtcgagttgatagagggccgcctgccggaggaaatggcttatcaatggaggtggcggccaggaggcgatgcactcaagtctagacgtgcggcaccgccaaaagatcttgcagacatgccaggatggaaacatgatccgaaattgtaa

SEQ ID NO: 175 - protein, 437 aa, Coniochaeta sp.
MTSNRADTRVIVVGGGGTIGSSTALHLVRSGYAPANITVLDTFEIPSAQSAGHDLNKIMGIDLRNKVDLQMSLEARQMWKEDELFQPFFHNTGRMDCEHTPEGIEKLKKLYQRLHDAGAGLEKTHAWLDNEDEILSKMPLLQRDQIQGWKAIWSQDGGWLAAAKAINAIGQFLKERGVKFGFGGAGSFKQPLFDDEGTTCIGVETADGTKYYADKVVLAAGAWSPTLVDLEDQCCSKAWVYAHIQLTPEEAAEYKGVPVVYNGEFGFFFEPDEFGVIKVCDEFPGFSRFKEHQPYGAPSPKRISVPRSHAKHPTDTYPDASEVSIKKAIATFLPRFQDKELFNRALCWCTDTADAALLMCEHPKWKNFILATGDSGHSFKILPNVGKYVVELIEGRLPEEMAYQWRWRPGGDALKSRRAAPPKDLADMPGWKHDPKL

SEQ ID NO: 176 - DNA, 1314 bp, Coniochaeta sp.
atgacgtcgaatcgtgcagatacaagggtgattgtcgtcggtggcggaggaacgattggttcctcgacagcgctgcatcttgtgaggagtggttatgctcccgcaaatatcacggtcttggacacatttgagattccatcggctcaatcagccggccatgatctcaacaagatcatgggaatagatctgcgcaacaaggtggacctgcaaatgagtctagaggctagacagatgtggaaggaggatgagttattccagcccttctttcacaataccggcagaatggactgcgaacacacgcctgagggtatcgagaaactgaaaaagctgtaccagcgtctgcacgatgccggtgcgggtctggagaagactcatgcctggttggacaacgaggatgagatcttatccaagatgccgttgcttcaacgtgaccaaatacaaggatggaaagcaatatggagtcaagatggcggctggttagctgcggcaaaggccatcaatgcgatcggacagttcttgaaagaacgtggtgtaaagttcggattcggcggcgctggatccttcaagcaaccccttttcgacgatgaaggcacaacttgcattggcgttgagacggcagatggtaccaaatattacgctgacaaggtggtcttagcagctggcgcatggagcccaaccctggtggacctggaagatcaatgttgctcgaaggcttgggtgtatgctcatattcagttgacgcctgaagaggccgctgagtataagggtgtcccagttgtgtataatggcgaatttggcttcttctttgagcctgatgagtttggtgtaataaaggtgtgcgacgagttcccaggattctcgcgcttcaaggaacatcaaccctatggcgccccatctccgaaacggatatcagtaccacgatcgcacgccaagcatcccacagacacttatccagacgcatccgaagtcagcatcaaaaaagcaatcgcgacgtttctccctcgatttcaggacaaggagctcttcaatcgcgccttgtgctggtgtacagacactgcggacgctgctctcttgatgtgtgaacaccccaaatggaagaatttcattctagcgaccggcgacagcggacactcattcaaaatcttgcctaacgtcggaaaatacgtagtcgagttgatagagggccgcctgccggaggaaatggcttatcaatggaggtggcggccaggaggcgatgcactcaagtctagacgtgcggcaccgccaaaagatcttgcagacatgccaggatggaaacatgatccgaaattgtaa

SEQ ID NO: 177 - protein, 437 aa, Coniochaeta sp.
MTSNRADTRVIVVGGGGTIGSSTALHLVRSGYAPANITVLDTFEIPSAQSAGHDLNKIMGIDARNKVDLQMSLEARQMWKEDELFQPFFHNTGRMDCEHTPEGIEKLKKLYQKLHDAGAGLEKTHAWLDNEDEILSKMPLLQRDQIQGWKAIWSQDGGWLAAAKAINAIGQFLKERGVKFGFGGAGSFKQPLFDDEGTTCIGVETADGTKYYADKVVLAAGAWSPTLVDLEDQCCSKAWVYAHIQLTPEEAAEYKGVPVVYNGEFGFFFEPDEFGVIKVCDEFPGFSRFKEHQPYGAPSPKRISVPRSHAKHPTDTYPDASEVSIKKAIATFLPRFQDKELFNRALCWCTDTADAALLMCEHPKWKNFILATGDSGHSFKILPNVGKYVVELIEGRLPEEMAYQWRWRPGGDALKSRRAAPPKDLADMPGWKHDPKL

SEQ ID NO: 178 - DNA, 1314 bp, Coniochaeta sp.
atgacgtcgaatcgtgcagatacaagggtgattgtcgtcggtggcggaggaacgattggttcctcgacagcgctgcatcttgtgaggagtggttatgctcccgcaaatatcacggtcttggacacatttgagattccatcggctcaatcagccggccatgatctcaacaagatcatgggaatagatgcgcgcaacaaggtggacctgcaaatgagtctagaggctagacagatgtggaaggaggatgagttattccagcccttctttcacaataccggcagaatggactgcgaacacacgcctgagggtatcgagaaactgaaaaagctgtaccagaaactgcacgatgccggtgcgggtctggagaagactcatgcctggttggacaacgaggatgagatcttatccaagatgccgttgcttcaacgtgaccaaatacaaggatggaaagcaatatggagtcaagatggcggctggttagctgcggcaaaggccatcaatgcgatcggacagttcttgaaagaacgtggtgtaaagttcggattcggcggcgctggatccttcaagcaaccccttttcgacgatgaaggcacaacttgcattggcgttgagacggcagatggtaccaaatattacgctgacaaggtggtcttagcagctggcgcatggagcccaaccctggtggacctggaagatcaatgttgctcgaaggcttgggtgtatgctcatattcagttgacgcctgaagaggccgctgagtataagggtgtcccagttgtgtataatggcgaatttggcttcttctttgagcctgatgagtttggtgtaataaaggtgtgcgacgagttcccaggattctcgcgcttcaaggaacatcaaccctatggcgccccatctccgaaacggatatcagtaccacgatcgcacgccaagcatcccacagacacttatccagacgcatccgaagtcagcatcaaaaaagcaatcgcgacgtttctccctcgatttcaggacaaggagctcttcaatcgcgccttgtgctggtgtacagacactgcggacgctgctctcttgatgtgtgaacaccccaaatggaagaatttcattctagcgaccggcgacagcggacactcattcaaaatcttgcctaacgtcggaaaatacgtagtcgagttgatagagggccgcctgccggaggaaatggcttatcaatggaggtggcggccaggaggcgatgcactcaagtctagacgtgcggcaccgccaaaagatcttgcagacatgccaggatggaaacatgatccgaaattgtaa

SEQ ID NO: 179 - protein, 437 aa, Coniochaeta sp.
MTSNRADTRVIVVGGGGTIGSSTALHLVRSGYAPANITVLDTFEIPSAQSAGHDLNKIMGIDHRNKVDLQMSLEARQMWKEDELFQPFFHNTGRMDCEHTPEGIEKLKKLYQKLHDAGAGLEKTHAWLDNEDEILSKMPLLQRDQIQGWKAIWSQDGGWLAAAKAINAIGQFLKERGVKFGFGGAGSFKQPLFDDEGTTCIGVETADGTKYYADKVVLAAGAWSPTLVDLEDQCCSKAWVYAHIQLTPEEAAEYKGVPVVYNGEFGFFFEPDEFGVIKVCDEFPGFSRFKEHQPYGAPSPKRISVPRSHAKHPTDTYPDASEVSIKKAIATFLPRFQDKELFNRALCWCTDTADAALLMCEHPKWKNFILATGDSGHSFKILPNVGKYVVELIEGRLPEEMAYQWRWRPGGDALKSRRAAPPKDLADMPGWKHDPKL

SEQ ID NO: 180 - DNA, 1314 bp, Coniochaeta sp.
atgacgtcgaatcgtgcagatacaagggtgattgtcgtcggtggcggaggaacgattggttcctcgacagcgctgcatcttgtgaggagtggttatgctcccgcaaatatcacggtcttggacacatttgagattccatcggctcaatcagccggccatgatctcaacaagatcatgggaatagatcatcgcaacaaggtggacctgcaaatgagtctagaggctagacagatgtggaaggaggatgagttattccagcccttctttcacaataccggcagaatggactgcgaacacacgcctgagggtatcgagaaactgaaaaagctgtaccagaaactgcacgatgccggtgcgggtctggagaagactcatgcctggttggacaacgaggatgagatcttatccaagatgccgttgcttcaacgtgaccaaatacaaggatggaaagcaatatggagtcaagatggcggctggttagctgcggcaaaggccatcaatgcgatcggacagttcttgaaagaacgtggtgtaaagttcggattcggcggcgctggatccttcaagcaaccccttttcgacgatgaaggcacaacttgcattggcgttgagacggcagatggtaccaaatattacgctgacaaggtggtcttagcagctggcgcatggagcccaaccctggtggacctggaagatcaatgttgctcgaaggcttgggtgtatgctcatattcagttgacgcctgaagaggccgctgagtataagggtgtcccagttgtgtataatggcgaatttggcttcttctttgagcctgatgagtttggtgtaataaaggtgtgcgacgagttcccaggattctcgcgcttcaaggaacatcaaccctatggcgccccatctccgaaacggatatcagtaccacgatcgcacgccaagcatcccacagacacttatccagacgcatccgaagtcagcatcaaaaaagcaatcgcgacgtttctccctcgatttcaggacaaggagctcttcaatcgcgccttgtgctggtgtacagacactgcggacgctgctctcttgatgtgtgaacaccccaaatggaagaatttcattctagcgaccggcgacagcggacactcattcaaaatcttgcctaacgtcggaaaatacgtagtcgagttgatagagggccgcctgccggaggaaatggcttatcaatggaggtggcggccaggaggcgatgcactcaagtctagacgtgcggcaccgccaaaagatcttgcagacatgccaggatggaaacatgatccgaaattgtaa

SEQ ID NO: 181 - protein, 437 aa, Coniochaeta sp.
MTSNRADTRVIVVGGGGTIGSSTALHLVRSGYAPANITVLDTFEIPSAQSAGHDLNKIMGIDHRNKVDLQMSLEARQMWKEDELFQPFFHNTGRMDCEHTPKGIEKLKKLYQKLHDAGAGLEKTHAWLDNEDEILSKMPLLQRDQIQGWKAIWSQDGGWLAAAKAINAIGQFLKERGVKFGFGGAGSFKQPLFDDEGTTCIGVETADGTKYYADKVVLAAGAWSPTLVDLEDQCCSKAWVYAHIQLTPEEAAEYKGVPVVYNGEFGFFFEPDEFGVIKVCDEFPGFSRFKEHQPYGAPSPKRISVPRSHAKHPTDTYPDASEVSIKKAIATFLPRFQDKELFNRALCWCTDTADAALLMCEHPKWKNFILATGDSGHSFKILPNVGKYVVELIEGRLPEEMAYQWRWRPGGDALKSRRAAPPKDLADMPGWKHDPKL

SEQ ID NO: 182 - DNA, 1314 bp, Coniochaeta sp.
atgacgtcgaatcgtgcagatacaagggtgattgtcgtcggtggcggaggaacgattggttcctcgacagcgctgcatcttgtgaggagtggttatgctcccgcaaatatcacggtcttggacacatttgagattccatcggctcaatcagccggccatgatctcaacaagatcatgggaatagatcatcgcaacaaggtggacctgcaaatgagtctagaggctagacagatgtggaaggaggatgagttattccagcccttctttcacaataccggcagaatggactgcgaacacacgcctaagggtatcgagaaactgaaaaagctgtaccagaaactgcacgatgccggtgcgggtctggagaagactcatgcctggttggacaacgaggatgagatcttatccaagatgccgttgcttcaacgtgaccaaatacaaggatggaaagcaatatggagtcaagatggcggctggttagctgcggcaaaggccatcaatgcgatcggacagttcttgaaagaacgtggtgtaaagttcggattcggcggcgctggatccttcaagcaaccccttttcgacgatgaaggcacaacttgcattggcgttgagacggcagatggtaccaaatattacgctgacaaggtggtcttagcagctggcgcatggagcccaaccctggtggacctggaagatcaatgttgctcgaaggcttgggtgtatgctcatattcagttgacgcctgaagaggccgctgagtataagggtgtcccagttgtgtataatggcgaatttggcttcttctttgagcctgatgagtttggtgtaataaaggtgtgcgacgagttcccaggattctcgcgcttcaaggaacatcaaccctatggcgccccatctccgaaacggatatcagtaccacgatcgcacgccaagcatcccacagacacttatccagacgcatccgaagtcagcatcaaaaaagcaatcgcgacgtttctccctcgatttcaggacaaggagctcttcaatcgcgccttgtgctggtgtacagacactgcggacgctgctctcttgatgtgtgaacaccccaaatggaagaatttcattctagcgaccggcgacagcggacactcattcaaaatcttgcctaacgtcggaaaatacgtagtcgagttgatagagggccgcctgccggaggaaatggcttatcaatggaggtggcggccaggaggcgatgcactcaagtctagacgtgcggcaccgccaaaagatcttgcagacatgccaggatggaaacatgatccgaaattgtaa

SEQ ID NO: 183 - protein, 437 aa, Coniochaeta sp.
MTSNRADTRVIVVGGGGTIGSSTALHLVRSGYAPANITVLDTFEIPSAQSAGHDLNKIMGIDHRNKVDLQMSLEARQMWKEDELFQPFFHNTGRMDCEHTPEGIEKLKKLYQKLHDAGAGLEKTHAWLDNEDEILSKMPLLQRDQIQGWKAIWSQDGGWLAAAKAINAIGQFLKERGVKFGFGGAGSFKQPLFDDEGTTCIGVETADGTKYYADKVVLAAGAWSPTLVDLEDQCCSKAWVYAHIQLTPEEAAEYKGVPVVYNGEFGFFFEPDEFGVIKVCDEFPGFSRFKEHQPYGAPSPKRISVPRSHAKHPTDTYPDASEVSIKKAIATFLPRFQDKELFNRALCWCTDTADAALLMCEHPKWKNFILATGDSGHSFKILPNVGKYVVELIEGRLPEEMAYQWRWRPGGDALKSRRKAPPKDLADMPGWKHDPKL

SEQ ID NO: 184 - DNA, 1314 bp, Coniochaeta sp.
atgacgtcgaatcgtgcagatacaagggtgattgtcgtcggtggcggaggaacgattggttcctcgacagcgctgcatcttgtgaggagtggttatgctcccgcaaatatcacggtcttggacacatttgagattccatcggctcaatcagccggccatgatctcaacaagatcatgggaatagatcatcgcaacaaggtggacctgcaaatgagtctagaggctagacagatgtggaaggaggatgagttattccagcccttctttcacaataccggcagaatggactgcgaacacacgcctgagggtatcgagaaactgaaaaagctgtaccagaaactgcacgatgccggtgcgggtctggagaagactcatgcctggttggacaacgaggatgagatcttatccaagatgccgttgcttcaacgtgaccaaatacaaggatggaaagcaatatggagtcaagatggcggctggttagctgcggcaaaggccatcaatgcgatcggacagttcttgaaagaacgtggtgtaaagttcggattcggcggcgctggatccttcaagcaaccccttttcgacgatgaaggcacaacttgcattggcgttgagacggcagatggtaccaaatattacgctgacaaggtggtcttagcagctggcgcatggagcccaaccctggtggacctggaagatcaatgttgctcgaaggcttgggtgtatgctcatattcagttgacgcctgaagaggccgctgagtataagggtgtcccagttgtgtataatggcgaatttggcttcttctttgagcctgatgagtttggtgtaataaaggtgtgcgacgagttcccaggattctcgcgcttcaaggaacatcaaccctatggcgccccatctccgaaacggatatcagtaccacgatcgcacgccaagcatcccacagacacttatccagacgcatccgaagtcagcatcaaaaaagcaatcgcgacgtttctccctcgatttcaggacaaggagctcttcaatcgcgccttgtgctggtgtacagacactgcggacgctgctctcttgatgtgtgaacaccccaaatggaagaatttcattctagcgaccggcgacagcggacactcattcaaaatcttgcctaacgtcggaaaatacgtagtcgagttgatagagggccgcctgccggaggaaatggcttatcaatggaggtggcggccaggaggcgatgcactcaagtctagacgtaaggcaccgccaaaagatcttgcagacatgccaggatggaaacatgatccgaaattgtaa

SEQ ID NO: 185 - protein, 438 aa, Aspergillus nidulans
MTPRANTKIIVVGGGGTMGSSTALHLLRAGYTPSNITVLDTCPIPSAQSAGYDLNKIMGIDHRNKPDLQLSLEALDMWKNDPLFKPFFHNVGMIDVSSTEKGIEKLRKLYQKLLDAGIGLEKTNFMLESEDEILAKAPHFTQEQIKGWKGLFCGDGGWLAAAKAINAIGQFLKEQGVKFGFGGAGTFKKPLFADAHEKTCIGVETVDGTKYYADKVVLAAGAWSSTLVDLEEQCVSKAWVFAHIQLTPAEAAAYKNTPVIYDGDYGFFFEPNENGIIKVCDEFPGFTHFKMHQPYGSPAPKPISVPRSHAKHPTDTYPHASEVTIKKAINRFLPRFNDKELFNRAMCWCTDTADSNLLVCEHPRWKGFYLATGDSGHSFKLLPNIGKHVVELLEERLESVFKDAWRWRPGSGDALKSRRAAPAKDLADMPGWRNEAKM

SEQ ID NO: 186 - DNA, 1317 bp, Aspergillus nidulans
atgacgccccgagccaacaccaaaatcattgtcgtcggcggcggcggcacaatgggctcgtcgacagccctacacctcctgcgcgccggctacacgccgtccaacattacagtgctcgacacgtgccctatcccctccgcacagtctgcaggctacgacctgaacaaaatcatgggcatcgatcatcgcaacaagcctgatttacagctctctcttgaggcgctggacatgtggaaaaatgatcctctcttcaagccgtttttccacaatgttggaatgatcgacgtctcttcaacagagaaaggcatcgagaaacttcggaagctgtaccagaaacttctcgacgcaggcattgggctcgagaagacgaatttcatgctggaaagtgaagacgagatcctggctaaagcgccgcatttcacgcaggagcagattaaaggctggaaaggcctgttctgtggcgacggcggctggctcgctgcagccaaagccatcaatgccattgggcagttcctcaaggaacagggcgtcaagtttggattcggcggcgccggcacgttcaaaaagccactcttcgccgatgcccacgagaagacgtgcatcggcgtcgagactgtagacggcacaaagtactacgccgacaaggtcgttctagcagctggtgcctggagttcgacgttggtcgatctggaggagcagtgcgtttcaaaggcctgggtctttgcccacatccaactgacgcccgctgaagcagccgcgtataagaacactcctgttatatacgacggtgactatgggtttttctttgagccgaatgaaaacggcatcataaaagtctgtgacgaattccctggcttcacgcatttcaaaatgcaccagccgtacggctcgccggcgcccaaacccatctctgtgcctcgttcccatgcgaagcaccccacagatacatacccgcacgcgtcggaggtcacgatcaaaaaggctatcaaccggttcctgccgaggttcaatgacaaggaactgtttaacagggccatgtgctggtgcaccgataccgcggatagcaatctgcttgtttgtgagcatccacgctggaaggggttttatcttgcaacaggggacagtgggcattcgttcaagttgctgccgaatattggaaagcatgttgtcgagttattggaggagaggctggaaagtgtgtttaaggatgcttggaggtggaggcctggcagtggggatgcattaaaaagtagacgggctgcgcctgcgaaggacctggcggatatgccggggtggaggaatgaggcaaagatgtag

SEQ ID NO: 187 - protein, 437 aa, Phaeosphaeria nodorum
MAPSRANTSVIVVGGGGTIGSSTALHLVRSGYTPSNVTVLDAYPIPSSQSAGNDLNKIMGVDHRNPVDLQLALEARQMWNEDELFKKFFHNTGRLDCAHGEKDIAKLKSLYQKLVDAGLDATNEWLDSEDEILKRMPLLSRDQIKGWKAIFSKDGGWLAAAKAINAVGEYLRDQGVRFGFYGAGSFKAPLLAEGVCIGVETVDGTRYYADKVVLAAGAWSPTLVELHEQCVSKAWVYGHIQLTPEEAARYKNSPVVYNGDVGFFFEPNEHGVIKVCDEFPGFTRFKMHQPFGAKAPKRISVPRSHAKHPTDTIPDASDVSIRRAIATFMPQFKNKKMFNQAMCWCTDTADSALLICEHPEWKNFVLATGDSGHSFKLLPNIGKHVVELLEGTLADDLAHAWRWRPGSGDALKSRRSAPAKDLADMPGWNHDKPRANL

SEQ ID NO: 188 - DNA, 1314 bp, Phaeosphaeria nodorum
atggccccgtcgcgtgctaatacgtcggtcattgtggttggtggtggtggtacgattggctcatctacggctctgcatctggtccgctcaggctataccccgtcgaacgtgacggttctggatgcatacccgattccgagctctcagagcgctggcaacgacctgaataaaatcatgggtgtcgatcatcgtaatccggtggatctgcagctggctctggaagcgcgccaaatgtggaacgaagacgaactgttcaagaagtttttccataacaccggccgtctggattgcgcgcacggtgaaaaagatattgccaaactgaagagcctgtatcagaaactggtggatgcgggtctggacgccacgaacgaatggctggatagtgaagacgaaatcctgaaacgtatgccgctgctgtcccgcgatcaaattaaaggctggaaggcgatcttttcaaaagacggtggttggctggcagcagcaaaggcaattaatgcagttggtgaatatctgcgtgatcagggcgtccgcttcggtttttacggcgccggttctttcaaagcaccgctgctggctgaaggcgtctgcatcggtgtcgaaaccgtggatggcacgcgctattacgcagacaaagtggttctggctgcaggtgcatggtcgccgaccctggttgaactgcatgaacagtgtgtgagcaaagcgtgggtttacggccacattcaactgacgccggaagaagccgcacgttataagaacagcccggtcgtgtacaatggcgatgtgggctttttctttgaaccgaacgaacatggcgttatcaaagtctgcgatgaatttccgggttttacccgcttcaagatgcaccagccgtttggtgccaaagcaccgaagcgtattagtgtgccgcgctcccatgccaaacacccgaccgatacgatcccggatgcaagtgacgtttccattcgtcgcgctatcgcgacctttatgccgcagttcaagaacaaaaagatgttcaaccaagcgatgtgctggtgtaccgatacggccgacagcgcgctgctgatttgtgaacatccggaatggaaaaactttgttctggcgaccggcgattcaggtcattcgttcaaactgctgccgaatatcggcaagcacgttgtcgaactgctggagggtacgctggcagatgacctggcacacgcatggcgttggcgtccgggtagtggtgatgcactgaaaagccgtcgctctgctccggcgaaagacctggctgatatgccgggctggaaccatgacaaaccgcgtgctaatctgtaa

SEQ ID NO: 189 - protein, 443 aa, Cryptococcus neoformans
MPPSRASTKVIVIGGGGTLGSSTALHLLRAGYTPSNITVLDTYLIPSAQSAGNDLNKIMGIDIRNPVDKQLSLEARDMWRNDEVFKPYFHNTGRLDCAHTPESIAKLRKLYEKILKAGSGLEKTHHWLSTEDEILARAPLLDRKQIKGWKAIYSEDGGWLAAAKAINSIGQVLKEKGVTFGFGSAGSFKKPLFDEDGTKAIGIETVDGTQYFADKVVLAAGAWSPTLVDLEGQCCSKAWVYAHMQLTPEEAAEYKECPVVYNSELGFFFEPNEKGVIKVCDEFPGFTRFKQHQPYGASSTKHISFPRSHAKHPTDTIPDESDASIRRAISAFLPRFKEKELFNRALCWCTDTADANLLICEHPKWKNFILATGDSGHSFKILPNIGKHVVELIEGTLAEDLAESWRWRPGSGDPLISRRAAPARDLADLPGWNHDEPSDDDMD

SEQ ID NO: 190 - DNA, 1332 bp, Cryptococcus neoformans
atgccgccgtcccgtgcttcaacgaaagtgattgtcattggtggtggtggtacgctgggctcctcaaccgccctgcatctgctgcgcgcgggctataccccgagtaacattaccgtgctggatacgtacctgatcccgagtgcccagtccgcaggcaacgacctgaataaaattatgggtattgatatccgcaatccggtggataaacaactgagcctggaagcccgtgatatgtggcgcaacgacgaagttttcaaaccgtacttccataacaccggtcgtctggactgcgctcacacgccggaatcaattgcgaaactgcgtaaactgtacgaaaaaatcctgaaagcaggctcaggtctggaaaaaacccatcactggctgtcgacggaagatgaaatcctggcacgtgcaccgctgctggaccgtaaacagattaaaggttggaaagcaatctatagtgaagatggcggttggctggcggccgcaaaagctattaactccatcggccaagtcctgaaagaaaaaggtgtgaccttcggctttggtagcgcaggctcttttaaaaaaccgctgttcgatgaagacggcacgaaagccattggtatcgaaaccgttgatggtacgcagtattttgccgacaaagtggttctggctgcaggtgcatggagcccgaccctggttgatctggaaggccagtgctgttctaaagcttgggtctacgcgcacatgcaactgacgccggaagaagccgcagaatataaagaatgcccggtcgtgtacaacagcgaactgggctttttctttgaaccgaacgaaaaaggtgtgatcaaagtttgtgatgaattcccgggctttacccgtttcaaacagcatcaaccgtacggtgctagctctacgaaacacattagctttccgcgctctcatgcgaaacacccgaccgatacgatcccggatgaaagtgacgcctccattcgtcgcgctatctctgcgtttctgccgcgtttcaaagaaaaagaactgtttaaccgcgcgctgtgctggtgtaccgatacggctgacgcgaacctgctgatttgtgaacacccgaaatggaaaaattttatcctggccaccggcgattcaggtcattcgttcaaaattctgccgaatatcggcaaacacgttgtcgaactgattgaaggtaccctggccgaagatctggcagaaagctggcgttggcgtccgggcagtggtgacccgctgatctcccgtcgcgctgcgccggcgcgcgacctggcggacctgccgggctggaaccacgacgaaccgagcgacgatgacatggactga

SEQ ID NO: 191 - protein, 440 aa, Curvularia clavata
MAPSRANTSVIVVGGGGTIGSSTALHLVRSGYTPSNITVLDAYPIPSSQSAGNDLNKIMGIDHRNKVDLQLSLEARQMWREDDLFKEYFHNTGRLDCAHGEEGLAKLRQLYQKLLDANAGLEETTEWLDSEDEILKKMPLLSRDQIKGWKAVYSQDGGWLAAAKAINAIGEYLRAQGVKFGFGGAGSFKQPLLAEGVCIGVETVDGTRYYADKVVLAAGAWSPTLVELHEQCVSKAWVYGHIQLTPEEAAEYKNSPVVYNGDVGFFFEPNEHGVIKVCDEFPGFTRFKMHQPFGAKAPKRISVPRSHAKHPTDTIPDASEKSIRKAIATFLPKFTEKELFNRHLCWCTDTADSALLICEHPEWKNFVLATGDSGHSFKLLPNIGKHVVELLEGTLADDLAHAWRWRPGSGDALKSRRSAPAKDLADMPGWKHDDVVKSKL

SEQ ID NO: 192 - DNA, 1323 bp, Curvularia clavata
atggccccgtcgcgtgctaatacgtcggtcattgtggttggtggtggtggtacgattggctcatctacggctctgcatctggtccgctcaggctataccccgtcgaacattacggttctggatgcatacccgattccgagctctcagagcgctggcaacgacctgaataaaatcatgggtatcgatcatcgtaataaggtggatctgcagctgtctctggaagcgcgccaaatgtggcgcgaagacgatctgttcaaggagtatttccataacaccggccgtctggattgcgcgcacggtgaagaaggtcttgccaaactgcgtcaactgtatcagaaactgctggatgcgaatgcgggtctggaagagacgaccgaatggctggatagtgaagacgaaatcctgaaaaaaatgccgctgctgtcccgcgatcaaattaaaggctggaaggcggtgtattcacaggacggtggttggctggcagcagcaaaggcaattaatgcaattggtgaatatctgcgtgctcagggcgtcaaattcggttttggcggcgccggttctttcaaacaaccgctgctggctgaaggcgtctgcatcggtgtcgaaaccgtggatggcacgcgctattacgcagacaaagtggttctggctgcaggtgcatggtcgccgaccctggttgaactgcatgaacagtgtgtgagcaaagcgtgggtttacggccacattcaactgacgccggaagaagccgcagaatataagaacagcccggtcgtgtacaatggcgatgtgggctttttctttgaaccgaacgaacatggcgttatcaaagtctgcgatgaatttccgggttttacccgcttcaagatgcaccagccgtttggtgccaaagcaccgaagcgtattagtgtgccgcgctcccatgccaaacacccgaccgatacgatcccggatgcaagtgaaaaatccattcgtaaagctatcgcgacctttctgccgaagttcacggagaaagagctgttcaaccgtcatctgtgctggtgtaccgatacggccgacagcgcgctgctgatttgtgaacatccggaatggaaaaactttgttctggcgaccggcgattcaggtcattcgttcaaactgctgccgaatatcggcaagcacgttgtcgaactgctggagggtacgctggcagatgacctggcacacgcatggcgttggcgtccgggtagtggtgatgcactgaaaagccgtcgctctgctccggcgaaagacctggctgatatgccgggctggaaacatgacgatgtggtgaaaagcaaactgtaa

SEQ ID NO: 193 - DNA, 28 bp, Artificial
  primer
caccttgttgcgatgatctattcccatg

SEQ ID NO: 194 - DNA, 28 bp, Artificial
  primer
cgcaacaaggtgaacctgcaaatgagtc

SEQ ID NO: 195 - DNA, 28 bp, Artificial
  primer
agagtccgcagtgtctgtacaccagcac

SEQ ID NO: 196 - DNA, 30 bp, Artificial
  primer
acactgcggactctactctcttgatgtgtg

SEQ ID NO: 197 - DNA, 10 bp, Artificial
  primer
aaaaaaaaaa

SEQ ID NO: 198 - DNA, 10 bp, Artificial
  primer
cccccccccc

SEQ ID NO: 199 - protein, 434 aa, Coniochaeta sp. NISL 9330
MTSNRADTRVIVVGGGGTIGSSTALHLVRSGYAPANITVLDTFPIPSAQSAGHDLNKIMGIDHRNKVNLQMSLEARQMWKEDELFQPFFHNTGRMDCEHTPKGIEKLKKLYQKLHDAGAGLEKTHAWLDNEDAILSKMPLLQRDQIQGWKAIWSQDGGWLAAAKAINAIGQFLKERGVKFGFGGAGSFKQPLFDDEGTTCIGVETADGTKYYADKVVLAAGAWSPTLVDLEDQCCSKAWVYAHIQLTPEEAAKYKGCPVVYHGEFGFFFEPDEFGVIKVCDEFPGFSRFKEHQPYGAPSPKRISVPRSHAKHPTDTYPDASEVSIKKAIATFLPRFKDKPLFNRALCWCTDTADSALLMCEHPKWKNFILATGDSGHSFKILPNVGKYVVELIEGRLPEEMAYQWRWRPGGDALKSRRAAPPKDLADMPGWKHD

SEQ ID NO: 200 - DNA, 1305 bp, Coniochaeta sp. NISL 9330
atgacctcaaaccgtgctgatacccgtgttattgttgttggtggtggtggtacgattggctcctcgaccgctctgcatctggtgcgtagtggctatgctccggcgaacattaccgtcctggatacgtttccgatcccgagcgcccagtctgcaggccatgatctgaataaaattatgggtatcgaccaccgtaacaaagttaatctgcagatgagcctggaagcgcgccaaatgtggaaagaagatgaactgttccagccgtttttccataacaccggccgtatggactgcgaacacacgccgaaaggtatcgaaaaactgaaaaaactgtaccaaaaactgcatgatgccggcgcaggtctggaaaaaacccacgcctggctggataacgaagacgcaattctgagcaaaatgccgctgctgcagcgtgatcagattcaaggttggaaagccatctggtctcaagacggcggttggctggcagcagcaaaagctattaatgcgatcggccagtttctgaaagaacgcggcgtgaaattcggttttggcggtgcaggttcttttaaacaaccgctgttcgatgacgaaggcaccacgtgtatcggtgttgaaaccgctgatggcacgaaatattacgcggacaaagtggttctggctgcaggtgcatggagtccgaccctggtcgatctggaagaccagtgctgttccaaagcgtgggtgtatgcgcatattcaactgacgccggaagaagccgcaaaatataaaggctgcccggtcgtgtaccacggcgaatttggctttttctttgaaccggatgaatttggcgtgatcaaagtttgtgacgaatttccgggtttttcacgtttcaaagaacatcagccgtatggtgcgccgtcgccgaaacgtattagcgttccgcgctctcatgccaaacacccgaccgatacgtacccggacgcaagtgaagtctccattaagaaagcgatcgcgacctttctgccgcgtttcaaagataaaccgctgtttaatcgcgcactgtgctggtgtaccgatacggccgacagcgcactgctgatgtgcgaacatccgaaatggaaaaactttattctggcgaccggcgattcaggtcactcgttcaaaatcctgccgaatgtgggcaaatatgttgtcgaactgattgaaggtcgcctgccggaagaaatggcttaccagtggcgttggcgtccgggcggtgatgccctgaaaagtcgccgtgctgctccgccgaaagacctggctgatatgccgggctggaaacatgactaa

SEQ ID NO: 201 - DNA, 30 bp, Artificial
  primer
gctgtcggccgtatcggtacaccagcacag

SEQ ID NO: 202 - DNA, 30 bp, Artificial
  primer
atacggccgacagcacactgctgatgtgcg

SEQ ID NO: 203 - protein, 434 aa, Coniochaeta sp.
MTSNRADTRVIVVGGGGTIGSSTALHLVRSGYAPANITVLDTFPIPSAQSAGHDLNKIMGIDHRNKVNLQMSLEARQMWKEDELFQPFFHNTGRMDCEHTPKGIEKLKKLYQKLHDAGAGLEKTHAWLDNEDAILSKMPLLQRDQIQGWKAIWSQDGGWLAAAKAINAIGQFLKERGVKFGFGGAGSFKQPLFDDEGTTCIGVETADGTKYYADKVVLAAGAWSPTLVDLEDQCCSKAWVYAHIQLTPEEAAKYKGCPVVYHGEFGFFFEPDEFGVIKVCDEFPGFSRFKEHQPYGAPSPKRISVPRSHAKHPTDTYPDASEVSIKKAIATFLPRFKDKPLFNRALCWCTDTADSTLLMCEHPKWKNFILATGDSGHSFKILPNVGKYVVELIEGRLPEEMAYQWRWRPGGDALKSRRAAPPKDLADMPGWKHD

SEQ ID NO: 204 - DNA, 1305 bp, Coniochaeta sp.
atgacctcaaaccgtgctgatacccgtgttattgttgttggtggtggtggtacgattggctcctcgaccgctctgcatctggtgcgtagtggctatgctccggcgaacattaccgtcctggatacgtttccgatcccgagcgcccagtctgcaggccatgatctgaataaaattatgggtatcgaccaccgtaacaaagttaatctgcagatgagcctggaagcgcgccaaatgtggaaagaagatgaactgttccagccgtttttccataacaccggccgtatggactgcgaacacacgccgaaaggtatcgaaaaactgaaaaaactgtaccaaaaactgcatgatgccggcgcaggtctggaaaaaacccacgcctggctggataacgaagacgcaattctgagcaaaatgccgctgctgcagcgtgatcagattcaaggttggaaagccatctggtctcaagacggcggttggctggcagcagcaaaagctattaatgcgatcggccagtttctgaaagaacgcggcgtgaaattcggttttggcggtgcaggttcttttaaacaaccgctgttcgatgacgaaggcaccacgtgtatcggtgttgaaaccgctgatggcacgaaatattacgcggacaaagtggttctggctgcaggtgcatggagtccgaccctggtcgatctggaagaccagtgctgttccaaagcgtgggtgtatgcgcatattcaactgacgccggaagaagccgcaaaatataaaggctgcccggtcgtgtaccacggcgaatttggctttttctttgaaccggatgaatttggcgtgatcaaagtttgtgacgaatttccgggtttttcacgtttcaaagaacatcagccgtatggtgcgccgtcgccgaaacgtattagcgttccgcgctctcatgccaaacacccgaccgatacgtacccggacgcaagtgaagtctccattaagaaagcgatcgcgacctttctgccgcgtttcaaagataaaccgctgtttaatcgcgcactgtgctggtgtaccgatacggccgacagcacactgctgatgtgcgaacatccgaaatggaaaaactttattctggcgaccggcgattcaggtcactcgttcaaaatcctgccgaatgtgggcaaatatgttgtcgaactgattgaaggtcgcctgccggaagaaatggcttaccagtggcgttggcgtccgggcggtgatgccctgaaaagtcgccgtgctgctccgccgaaagacctggctgatatgccgggctggaaacatgactaa

SEQ ID NO: 205 - DNA, 27 bp, Artificial
  primer
atgatctattcccatgatcttgttgag

SEQ ID NO: 206 - DNA, 30 bp, Artificial
  primer
tgggaatagatcatggcaacaaggtgaacc

SEQ ID NO: 207 - DNA, 30 bp, Artificial
  primer
gtggtcgatacccataattttattcagatc

SEQ ID NO: 208 - DNA, 30 bp, Artificial
  primer
tgggtatcgaccacggtaacaaagttaatc

SEQ ID NO: 209 - protein, 437 aa, Coniochaeta sp.
MTSNRADTRVIVVGGGGTIGSSTALHLVRSGYAPANITVLDTFEIPSAQSAGHDLNKIMGIDHRNKVNLQMSLEARQMWKEDELFQPFFHNTGRMDCEHTPKGIEKLKKLYQKLHDAGAGLEKTHAWLDNEDEILSKMPLLQRDQIQGWKAIWSQDGGWLAAAKAINAIGQFLKERGVKFGFGGAGSFKQPLFDDEGTTCIGVETADGTKYYADKVVLAAGAWSPTLVDLEDQCCSKAWVYAHIQLTPEEAAEYKGVPVVYNGEFGFFFEPDEFGVIKVCDEFPGFSRFKEHQPYGAPSPKRISVPRSHAKHPTDTYPDASEVSIKKAIATFLPRFQDKELFNRALCWCTDTADSTLLMCEHPKWKNFILATGDSGHSFKILPNVGKYVVELIEGRLPEEMAYQWRWRPGGDALKSRRAAPPKDLADMPGWKHDPKL

SEQ ID NO: 210 - DNA, 1314 bp, Coniochaeta sp.
atgacgtcgaatcgtgcagatacaagggtgattgtcgtcggtggcggaggaacgattggttcctcgacagcgctgcatcttgtgaggagtggttatgctcccgcaaatatcacggtcttggacacatttgagattccatcggctcaatcagccggccatgatctcaacaagatcatgggaatagatcatcgcaacaaggtgaacctgcaaatgagtctagaggctagacagatgtggaaggaggatgagttattccagcccttctttcacaataccggcagaatggactgcgaacacacgcctaagggtatcgagaaactgaaaaagctgtaccagaaactgcacgatgccggtgcgggtctggagaagactcatgcctggttggacaacgaggatgagatcttatccaagatgccgttgcttcaacgtgaccaaatacaaggatggaaagcaatatggagtcaagatggcggctggttagctgcggcaaaggccatcaatgcgatcggacagttcttgaaagaacgtggtgtaaagttcggattcggcggcgctggatccttcaagcaaccccttttcgacgatgaaggcacaacttgcattggcgttgagacggcagatggtaccaaatattacgctgacaaggtggtcttagcagctggcgcatggagcccaaccctggtggacctggaagatcaatgttgctcgaaggcttgggtgtatgctcatattcagttgacgcctgaagaggccgctgagtataagggtgtcccagttgtgtataatggcgaatttggcttcttctttgagcctgatgagtttggtgtaataaaggtgtgcgacgagttcccaggattctcgcgcttcaaggaacatcaaccctatggcgccccatctccgaaacggatatcagtaccacgatcgcacgccaagcatcccacagacacttatccagacgcatccgaagtcagcatcaaaaaagcaatcgcgacgtttctccctcgatttcaggacaaggagctcttcaatcgcgccttgtgctggtgtacagacactgcggactctactctcttgatgtgtgaacaccccaaatggaagaatttcattctagcgaccggcgacagcggacactcattcaaaatcttgcctaacgtcggaaaatacgtagtcgagttgatagagggccgcctgccggaggaaatggcttatcaatggaggtggcggccaggaggcgatgcactcaagtctagacgtgcggcaccgccaaaagatcttgcagacatgccaggatggaaacatgatccgaaattgtaa

SEQ ID NO: 211 - protein, 437 aa, Coniochaeta sp.
MTSNRADTRVIVVGGGGTIGSSTALHLVRSGYAPANITVLDTFEIPSAQSAGHDLNKIMGIDHGNKVNLQMSLEARQMWKEDELFQPFFHNTGRMDCEHTPKGIEKLKKLYQKLHDAGAGLEKTHAWLDNEDEILSKMPLLQRDQIQGWKAIWSQDGGWLAAAKAINAIGQFLKERGVKFGFGGAGSFKQPLFDDEGTTCIGVETADGTKYYADKVVLAAGAWSPTLVDLEDQCCSKAWVYAHIQLTPEEAAEYKGVPVVYNGEFGFFFEPDEFGVIKVCDEFPGFSRFKEHQPYGAPSPKRISVPRSHAKHPTDTYPDASEVSIKKAIATFLPRFQDKELFNRALCWCTDTADSTLLMCEHPKWKNFILATGDSGHSFKILPNVGKYVVELIEGRLPEEMAYQWRWRPGGDALKSRRAAPPKDLADMPGWKHDPKL

SEQ ID NO: 212 - DNA, 1314 bp, Coniochaeta sp.
atgacgtcgaatcgtgcagatacaagggtgattgtcgtcggtggcggaggaacgattggttcctcgacagcgctgcatcttgtgaggagtggttatgctcccgcaaatatcacggtcttggacacatttgagattccatcggctcaatcagccggccatgatctcaacaagatcatgggaatagatcatggcaacaaggtgaacctgcaaatgagtctagaggctagacagatgtggaaggaggatgagttattccagcccttctttcacaataccggcagaatggactgcgaacacacgcctaagggtatcgagaaactgaaaaagctgtaccagaaactgcacgatgccggtgcgggtctggagaagactcatgcctggttggacaacgaggatgagatcttatccaagatgccgttgcttcaacgtgaccaaatacaaggatggaaagcaatatggagtcaagatggcggctggttagctgcggcaaaggccatcaatgcgatcggacagttcttgaaagaacgtggtgtaaagttcggattcggcggcgctggatccttcaagcaaccccttttcgacgatgaaggcacaacttgcattggcgttgagacggcagatggtaccaaatattacgctgacaaggtggtcttagcagctggcgcatggagcccaaccctggtggacctggaagatcaatgttgctcgaaggcttgggtgtatgctcatattcagttgacgcctgaagaggccgctgagtataagggtgtcccagttgtgtataatggcgaatttggcttcttctttgagcctgatgagtttggtgtaataaaggtgtgcgacgagttcccaggattctcgcgcttcaaggaacatcaaccctatggcgccccatctccgaaacggatatcagtaccacgatcgcacgccaagcatcccacagacacttatccagacgcatccgaagtcagcatcaaaaaagcaatcgcgacgtttctccctcgatttcaggacaaggagctcttcaatcgcgccttgtgctggtgtacagacactgcggactctactctcttgatgtgtgaacaccccaaatggaagaatttcattctagcgaccggcgacagcggacactcattcaaaatcttgcctaacgtcggaaaatacgtagtcgagttgatagagggccgcctgccggaggaaatggcttatcaatggaggtggcggccaggaggcgatgcactcaagtctagacgtgcggcaccgccaaaagatcttgcagacatgccaggatggaaacatgatccgaaattgtaa

SEQ ID NO: 213 - protein, 434 aa, Coniochaeta sp.
MTSNRADTRVIVVGGGGTIGSSTALHLVRSGYAPANITVLDTFPIPSAQSAGHDLNKIMGIDHGNKVNLQMSLEARQMWKEDELFQPFFHNTGRMDCEHTPKGIEKLKKLYQKLHDAGAGLEKTHAWLDNEDAILSKMPLLQRDQIQGWKAIWSQDGGWLAAAKAINAIGQFLKERGVKFGFGGAGSFKQPLFDDEGTTCIGVETADGTKYYADKVVLAAGAWSPTLVDLEDQCCSKAWVYAHIQLTPEEAAKYKGCPVVYHGEFGFFFEPDEFGVIKVCDEFPGFSRFKEHQPYGAPSPKRISVPRSHAKHPTDTYPDASEVSIKKAIATFLPRFKDKPLFNRALCWCTDTADSTLLMCEHPKWKNFILATGDSGHSFKILPNVGKYVVELIEGRLPEEMAYQWRWRPGGDALKSRRAAPPKDLADMPGWKHD

SEQ ID NO: 214 - DNA, 1305 bp, Coniochaeta sp.
atgacctcaaaccgtgctgatacccgtgttattgttgttggtggtggtggtacgattggctcctcgaccgctctgcatctggtgcgtagtggctatgctccggcgaacattaccgtcctggatacgtttccgatcccgagcgcccagtctgcaggccatgatctgaataaaattatgggtatcgaccacggtaacaaagttaatctgcagatgagcctggaagcgcgccaaatgtggaaagaagatgaactgttccagccgtttttccataacaccggccgtatggactgcgaacacacgccgaaaggtatcgaaaaactgaaaaaactgtaccaaaaactgcatgatgccggcgcaggtctggaaaaaacccacgcctggctggataacgaagacgcaattctgagcaaaatgccgctgctgcagcgtgatcagattcaaggttggaaagccatctggtctcaagacggcggttggctggcagcagcaaaagctattaatgcgatcggccagtttctgaaagaacgcggcgtgaaattcggttttggcggtgcaggttcttttaaacaaccgctgttcgatgacgaaggcaccacgtgtatcggtgttgaaaccgctgatggcacgaaatattacgcggacaaagtggttctggctgcaggtgcatggagtccgaccctggtcgatctggaagaccagtgctgttccaaagcgtgggtgtatgcgcatattcaactgacgccggaagaagccgcaaaatataaaggctgcccggtcgtgtaccacggcgaatttggctttttctttgaaccggatgaatttggcgtgatcaaagtttgtgacgaatttccgggtttttcacgtttcaaagaacatcagccgtatggtgcgccgtcgccgaaacgtattagcgttccgcgctctcatgccaaacacccgaccgatacgtacccggacgcaagtgaagtctccattaagaaagcgatcgcgacctttctgccgcgtttcaaagataaaccgctgtttaatcgcgcactgtgctggtgtaccgatacggccgacagcacactgctgatgtgcgaacatccgaaatggaaaaactttattctggcgaccggcgattcaggtcactcgttcaaaatcctgccgaatgtgggcaaatatgttgtcgaactgattgaaggtcgcctgccggaagaaatggcttaccagtggcgttggcgtccgggcggtgatgccctgaaaagtcgccgtgctgctccgccgaaagacctggctgatatgccgggctggaaacatgactaa

SEQ ID NO: 215 - DNA, 30 bp, Artificial
  primer
tgggaatagatcatgccaacaaggtgaacc

SEQ ID NO: 216 - DNA, 30 bp, Artificial
  primer
tgggaatagatcatgtcaacaaggtgaacc

SEQ ID NO: 217 - DNA, 30 bp, Artificial
  primer
tgggaatagatcatatcaacaaggtgaacc

SEQ ID NO: 218 - DNA, 30 bp, Artificial
  primer
tgggaatagatcatctgaacaaggtgaacc

SEQ ID NO: 219 - DNA, 30 bp, Artificial
  primer
tgggaatagatcatatgaacaaggtgaacc

SEQ ID NO: 220 - DNA, 30 bp, Artificial
  primer
tgggaatagatcatagcaacaaggtgaacc

SEQ ID NO: 221 - DNA, 30 bp, Artificial
  primer
tgggaatagatcataccaacaaggtgaacc

SEQ ID NO: 222 - DNA, 30 bp, Artificial
  primer
ctttttcagtttctcgatacccttaggcgt

SEQ ID NO: 223 - DNA, 30 bp, Artificial
  primer
agaaactgaaaaagtattaccagaaactgc

SEQ ID NO: 224 - DNA, 30 bp, Artificial
  primer
agaaactgaaaaagttttaccagaaactgc

SEQ ID NO: 225 - DNA, 30 bp, Artificial
  primer
agaaactgaaaaagcattaccagaaactgc

SEQ ID NO: 226 - DNA, 30 bp, Artificial
  primer
ttcgcagtccattctgccggtattgtgaaa

SEQ ID NO: 227 - DNA, 30 bp, Artificial
  primer
atggactgcgaaagcacgcctaagggtatc

SEQ ID NO: 228 - DNA, 30 bp, Artificial
  primer
atgatcgacacccatgattttattcaggtc

SEQ ID NO: 229 - DNA, 30 bp, Artificial
  primer
agtaatccggtggatctgcagctggctctg

SEQ ID NO: 230 - DNA, 30 bp, Artificial
  primer
atcgatacccataattttattcaggtcgtt

SEQ ID NO: 231 - DNA, 30 bp, Artificial
  primer
catcgcaataaagttgatctgcaactgagc

SEQ ID NO: 232 - DNA, 22 bp, Artificial
  primer
aattctgtttcctgtgtgaaat

SEQ ID NO: 233 - DNA, 30 bp, Artificial
  primer
aagcttggctgttttggcggatgagagaag

SEQ ID NO: 234 - DNA, 35 bp, Artificial
  primer
aaaacagccaagctttcagcgtgattccgagtctt

SEQ ID NO: 235 - DNA, 34 bp, Artificial
  primer
aggaaacagaattcatgacgaccccgcgtaaaga

SEQ ID NO: 236 - DNA, 30 bp, Artificial
  primer
atgatcgatacccataattttattcaggtc

SEQ ID NO: 237 - DNA, 30 bp, Artificial
  primer
atgaataaagttgatctgcaactgagcctg

SEQ ID NO: 238 - DNA, 30 bp, Artificial
  primer
agcaataaagttgatctgcaactgagcctg

SEQ ID NO: 239 - DNA, 30 bp, Artificial
  primer
accaataaagttgatctgcaactgagcctg

SEQ ID NO: 240 - DNA, 1323 bp, Curvularia clavata
atggccccgagtcgcgctaacacgagcgtcattgtggtgggtggtggtggcacgattggttcctcaacggcactgcatctggtccgtagcggctataccccgtctaacattaccgtgctggacacgtacccgatcccgagcgcccagtctgcaggcaacgatctgaataaaattatgggtatccgtctgcgcaacaaagttgatctgcagctgtcactggaagcccgtcaaatgtggcgcgaagatgacctgtttaaagaatacttccataacaccggccgtctggattgcgcacacggtgaagaaggtctggccgacctgcgccaggcttaccaagcgctgctggatgccaacgcaggtctggaagaaaccacggaatggctggattcagaagacgaaattctgaagaaaatgccgctgctggatcgtgaacagatcaaaggttggaaagccgtgtattcgcaagatggcggttggctggcggccgcaaaagccattaatgcaatcggcgaatacctgcgcgcgcagggcgttaaattcggttttggcggtgctggttcctttaaacagccgctgctggcagaaggcgtctgcattggtgtcgaaaccgtggatggcacgcgttattacgcggacaaagtggttctggctgcaggtgcatggagtccggtgctggttgatctggaagaccagtgtgtgtccaaagcgtgggtttatgcgcatatccaactgaccccggaagaagccgcagaatataaaaacgtcccggtcgtgtacaatggcgatgtgggctttttctttgaaccggacgaacatggcgttattaaagtctgcgatgaatttccgggttttacccgcttcaaacagcaccaaccgtatggcgctaaagcgccgaaacgtatctcagtgccgcgttcggctgcaaaacacccgaccgatacgtacccggacgcgagtgaaaaatccattcgtaaagccatcgcaacctttctgccgaaattcacggaaaaagaactgtttaatcgccatctgtgctggtgtaccgatacggccgacgccgcactgctgatgtgtgaacacccggaatggaaaaactttgttctggcgaccggcgatagcggtcatacgttcaaactgctgccgaatattggcaaacacgttgtcgaactgctggaaggtaccctggcagaagacctggctcatgcgtggcgttggcgtccgggtacgggtgatgcactgaaatctcgtcgcgctgcgccggcgaaagacctggcggatatgccgggctggaaacacgacgatgtggtgaaaagcaaactgtaa

SEQ ID NO: 241 - DNA, 30 bp, Artificial
  primer
gatacccataattttattcagatcgttgcc

SEQ ID NO: 242 - DNA, 30 bp, Artificial
  primer
gatctgcgcaacaaagttgatctgcagctg

SEQ ID NO: 243 - DNA, 30 bp, Artificial
  primer
gatcatcgcaacaaagttgatctgcagctg

SEQ ID NO: 244 - DNA, 30 bp, Artificial
  primer
ggccagacctttttcaccgtgtgcgcaatc

SEQ ID NO: 245 - DNA, 30 bp, Artificial
  primer
aaactgcgccaggcttaccaagcgctgctg

SEQ ID NO: 246 - DNA, 30 bp, Artificial
  primer
atgatcgatacccataattttattcagatc

SEQ ID NO: 247 - DNA, 30 bp, Artificial
  primer
ctcaacaaagttgatctgcagctgtcactg

SEQ ID NO: 248 - DNA, 30 bp, Artificial
  primer
accaacaaagttgatctgcagctgtcactg